European Patent Specification EP 3 283 090 B1, published June 7, 2023. Title: ALGAL CHLOROPLASTIC SRP54 MUTANTS. Applicant: SYNTHETIC GENOMICS, INC. DIPETRILLO, Christen G. MCCARREN, Jay SORIAGA, Leah. The sequence listing filed with the application follows.

SEQUENCE LISTING (74 sequences)

SEQ ID NO: 1 - DNA, 1707 bp, Parachlorella sp.
  misc_feature: encodes cpSRP54
atgcttcggcagcagctgttgcacagcggcaggcagccgggtgcgacatgcagcttactaacctgctcgacatggcgaccgtctgccttgttcggccgtcctaagccccaaaaactgcacagccagcgcttgcagcatcagggccgcccctcccgcctcgtcgtgcgcagcgcaatgttcgacaacctgagccgcagcctggagagggcgtgggacatggtgcgcaaggacgggcggctaacggcggacaacatcaaggagcccatgcgggagattcgcagggcgctgcttgaggcggatgtgaggctgggggcgccgctgatcagattcttggtatctaccccccccccctcccaggtctccctccccgtggtgcgcaagtttgtgaaggcggtggaggagaaggcgctgggttctgcagtgaccaagggtgtcacccccgaccagcagctggtgaaggtggtgtacgaccagctgcgggagctgatgggggggcagcaggaagggctggtgcccacttcgccagaggagccgcaggtgatcttgatggcggggctgcagggcacggggaagacgacagctgcggggaagctggccttgttcctgcagaagaaggggcagaaggtgctgctggtggccaccgacatctaccgccccgccgccatcgaccagctggtgaagctgggcgacaggataggggtgccggtgttccagctgggaacccaggtgcagccgccggagattgcaaggcaggggctggagaaggcgcgagcagaggggtttgacgccgtcatcgtcgacacggcggggcggctgcagatcgaccagagcatgatggaggagctggtgcagatcaagtccacggtgaagccctccgacacgctgctagtggtcgatgcgatgacggggcaggaggcagccgggctggtgaaggcgttcaatgatgccgtggacatcacaggcgccgtgctgaccaagcttgacggggacagccgcggcggcgccgcgctgagcgtgcgccaggtcagcgggcggcccatcaagtttgtgggcatgggggagggcatggaggcgctggagcccttctaccccgagcgcatggccagcaggattctgggcatgggtgacgtggtcaccctggtggagaaggctgaggagagcatcaaggaagaggaggcgcaggagatatcgcggaagatgctgtcggccaaatttgactttgacgacttcctgaagcagtacaagatggtggcggggatggggaacatggcccaaatcatgaagatgctgccaggcatgaacaagtttacggagaagcagctggcgggcgttgagaagcagtacaaggtgtacgagagcatgatccagagcatgacggtgaaggagcgcaagcagccggagctgttggtgaagtcgccctccaggaggcggcgcatagcgcgcgggtcggggcgctcggagcgggaggtcacagagctgctgggggtgttcaccaacctgcggacgcagatgcagagcttctccaaaatgatggccatgggggggatgggcatgggctccatgatgagcgacgaggagatgatgcaggccacgctggcaggcgccggcccccgccccgtgccagctggcaaggtgcggcggaagaagctggccgcggcgggcgggtcgcggggcatggctgagctggcatccctgaaggcagaatga

SEQ ID NO: 2 - protein, 568 aa, Parachlorella sp.
  misc_feature: cpSRP54
MLRQQLLHSGRQPGATCSLLTCSTWRPSALFGRPKPQKLHSQRLQHQGRPSRLVVRSAMFDNLSRSLERAWDMVRKDGRLTADNIKEPMREIRRALLEADVRLGAPLIRFLVSTPPPSQVSLPVVRKFVKAVEEKALGSAVTKGVTPDQQLVKVVYDQLRELMGGQQEGLVPTSPEEPQVILMAGLQGTGKTTAAGKLALFLQKKGQKVLLVATDIYRPAAIDQLVKLGDRIGVPVFQLGTQVQPPEIARQGLEKARAEGFDAVIVDTAGRLQIDQSMMEELVQIKSTVKPSDTLLVVDAMTGQEAAGLVKAFNDAVDITGAVLTKLDGDSRGGAALSVRQVSGRPIKFVGMGEGMEALEPFYPERMASRILGMGDVVTLVEKAEESIKEEEAQEISRKMLSAKFDFDDFLKQYKMVAGMGNMAQIMKMLPGMNKFTEKQLAGVEKQYKVYESMIQSMTVKERKQPELLVKSPSRRRRIARGSGRSEREVTELLGVFTNLRTQMQSFSKMMAMGGMGMGSMMSDEEMMQATLAGAGPRPVPAGKVRRKKLAAAGGSRGMAELASLKAE

SEQ ID NO: 3 - protein, 549 aa, Chlamydomonas reinhardtii
  misc_feature: cpSRP54
MQTALRARSAAPRGACNRTAVAPVASAHLRGQYAPFSGAQARPALGRQRQQQQQQRRGALVIRSAMFDSLSRSIEKAQRLIGKSGTLTAENMKEPLKEVRRALLEADVSLPVVRRFIKKVEERALGTKVREGRAMGTKWKSVVNCPLQDGLGNRGVGRARTEVGHRAACVHGARGVGKTTAAGKLALYLKKAKKSCLLVATDVYRPAAIDQLVKLGAAIDVPVFEMGTDVSPVEIAKKGVEEARRLGVDAVIIDTAGRLQVDEGMMAELRDVKSAVRPSDTLLVVDAMTGQEAANLVRSFNEAVDISGAILTKMDGDSRGGAALSVREVSGKPIKFVGVGEKMEALEPFYPERMASRILGMGDVLTLYEKAEAAIKEEDAQKTMERLMEEKFDFNDFLNQWKAMNNMGGLQMLKMMPGFNKISEKQLYEAEKQFGVYEAIIGAMDEEERSNPEVLIKNLARRRRVAQDSGKSEAEVTKLMAAYTSMKAQVGGMSKLLKLQKAGADPQKANSLLQELVASAGKKVAPGKVRRKKEKEPLSKARGFGSSSK

SEQ ID NO: 4 - protein, 559 aa, Micromonas pusilla
  misc_feature: cpSRP54
MRHLLSSASIRQYDKWSLVSSHAKKPALVCASKHTKSAVKLQCTSRGSSNRTIQLLLFQQFRPAKRGKLLITRADSFGTLSERLNSAWSALKDEDDLSVENISLPLKDIRRALLEADVSLPVVRRFIKSVEEKSIGVKVTKGVSASQQLTKVVADELCELMGGFGGDKLIFRKEGEGPTVILMAGLQGVGKTTACGKLALFLKAQGKQSLLVATDVYRPAAIDQLKKLGEQIDVPVFELGTDFSPPDIARSGVEKAKLENFDVVIVDTAGRLQVDEMLMAELLATKAATRADETLLVVDAMTGQEAASLTAAFNDAVGITGAVLTKMDGDTRGGAALSVREVSGKPIKFIGSGEKLDALEPFFPERMTTRILGMGDVVSLVERAQVAVKEEQANLMRDKILSATFDFNDFLSQLEMMGKMGGMGGLTKMMPGMNTMSDKELQDAEKSLSVAKSLIMSMTPRERQFPDLLVAGSSAASRRGRVVEGSGRSDKDLANLIVMFGSMRVKMQSLSAQMNGTAKEVGLVPQLSEVDLNKLAFEGVGKRVSPGMVRRRKLNASFG

SEQ ID NO: 5 - protein, 568 aa, Micromonas sp.
  misc_feature: cpSRP54
MEARTKQARAPKGSIWCAQRARKDLRARGCRGLGSRISKGQPFSPLTLSTPAVTEIGFGTLLYGSRLSAGGSRRGETMLRRASAFGSLTERLNSVWATLKDEDDLSLENIKGPLKDIRRALLEADVSLPVVRRFIKNIEQKAIGTRVTKGVNAGQQLTKVVADELCELMGGFGGDSLAFKDPSMGPTVILMAGLQGVGKTTACGKLALYLKKQGKDSLLVATDVYRPAAIEQLKRLGEQVKTPVFDMGVRVDPPEVARLGLEKARAEGIDVVIIDTAGRLQVDVHLMEELRATKIATAADEILLVVDAMTGQEAAALTAAFDEAVGITGAVLTKMDGDTRGGAALSVREVSGKPIKFTGVGEKMEALEPFYPERMASRILGMGDVVTLVERAQQVVKNEEAEQMRDKILSATFDFNDFIKQMEMMGQMGGMDGFMKLLPGMSGMSEREMQEADKSLKVAKSLILSMTSKERQFPDILVAGASAKSRRKRIIEGAGRSEKDLSQLIVLFGSMRVKMQKMTAEITGASAEVGLTPQLSEEDMNTLANEGLRKNVSPGMVRRLRIRRLTGS

SEQ ID NO: 6 - protein, 481 aa, Paulinella chromatophora
  misc_feature: cpSRP54
MFDELSARFEEAVKSLKGLSAITENNVENALKQVRRALIEADVSLVVVKEFMEEVRSKSIGIEVVRGIKPDQKFIQVVYEQLIEIMGANNTPLHKQSHTVTVVLMAGLQGAGKTTAAAKLALYLKNQGEKVLMVAADVYRPAAIDQLFVLGKQIDVEVFTLNPESIPEDIAAAGLQKAIREGFDYLIVDTAGRLQIDTAMMQEMVRIRSAVNPNEILLVVDSMIGQEAAELTRAFHEQIGITGAVLTKLDGDARGGAALSIRKVSGAPIKFIGTGEKVEALQPFHPERMASRILGMGDIVTLVEKAQEEVELADVEKMQRKLQEASFDFSDFLQQMRLVKRMGSLGGLMKMIPGMNKIDSTMLREGEAQLKRIESMIGSMTPTEREKPELLASQPSRRGRIAKGSGHKIADVDKMLVDFQKMRGFMQQMTKGNNFANPLSMGANMFSQPNMTVPQTKISNTNESRMRNSRATKKKKGFGQL

SEQ ID NO: 7 - protein, 498 aa, Ostreococcus lucimarinus
  misc_feature: cpSRP54
MTRADAFAGMSDKLDKAWARLQGEKDLNADNVKAPLKDVRRALLEADVSLPVVRRFIARCEEKAVGMKVTKGVEPGQMLVKCVADELCELMGGVGAEGIKFRDDGEPTVVLMAGLQGVGKTTACGKLSLALRKQGKSVLLVATDVYRPAAIDQLKTLGKQIGVPVFDMGVDGNPPEIAARGVRKAKDEDIDVVIVDTAGRLNIDEKLMGELKATKEATSADETLLVVDAMTGQEAATLTASFNEAVEITGAILTKMDGDTRGGAALSVREVSGKPIKFTGVGEKMDALEPFYPERMTSRILGMGDIVSLVEKVQAGVKEEEAEKIKQKIMSATFDFNDFVGQLEMMNNMGGMKQIMQMMPGTAKLSEADMEAAGKSMTIAKSLINSMTKEERQYPDMLVASTTADSRRQRIVKGSGRTEADLAQLIMMFGGMRTQMQKMSGQLGGQAGDVGLQPQLSEAELSKLAMNKIRKTVKPGMVRRQKAKKVPKFLAERESFSQ

SEQ ID NO: 8 - protein, 426 aa, Ostreococcus tauri
  misc_feature: cpSRP54
MKVTKGVEPGQMLVKAVADELCELMGGVGAEGIKFRDDGEPTVILMAGLQGVGKTTACGKLSLAMRKQGKTVLLVATDVYRPAAIDQLKTLGTQIGVPVFDMGVDASPPEVAARGVRKAKEEDIDVVIVDTAGRLNIDEKLMSELKDTKLATKADETLLVVDAMTGQEAANLTASFQRGDGRRTRRGGAALSVARSFRKAHQFTASVKMDALEPFYPERMTSRILGMGDIVSLVEKVQSEVKEAEAEKLKEKILKATFDFNDFVTQLEMMNNMGSMKQIMQMLPGTTKLSESEMEAAEKSFKIARSLINSMTKEERQFPDMLVASTTAESRRARIVKGSGRTEADLAQLIIMFGSMRGKMQQLSGELGGEAGNVGLQPQLSAAELEKLTTNKLRKNIKPGMVRRLKSKKIPIAKNGDRMGISASAD

SEQ ID NO: 9 - protein, 510 aa, Volvox carteri
  misc_feature: cpSRP54
MSRPAALRGAGNRKLTATVTAAHLRGIAFTSIRTCQGAKGGSLGLPHPSPPLALPRRGRGRGAAVVVRAAMFDNLSKSLEKAQRLIGGCEVPGVGVVGKSGTLTAENMKEPLKEVRRALLEADVSLPVVRRFVKKVEERALGTKVIEGVTPDVQFIKVVSNELIELMGGGVGAKDLEPGFPQIILMAGLQGVGKTTAAGKLALYLKKAKKSCLLVATDVYRPAAIDQLVKLGAAIDVPVFELGTQVSGKPIKFVGVGEKMEALEPFYPERMASRILGMGDVLTLYEKAEAAIKEEDAKAVMDRLMEEKFDFNDFLNQWKSMNNMGGMQILKMMPGFNKERSNPEVIIKSLARRRRVAQDSGHSEAEVAKLMTAYTAMRTQVGGMSKLLKLQKSGGDPSQAEKLLKELVASAGKKVAPGKPPGDPAGSFISTPRTPHPPPGPLGPRSQVRRKKEKEPISKARGFGSPSNFNHDLSPPGSSPAAYTYTLSRLSCQRLCDGGGLLDDWNLWRR

SEQ ID NO: 10 - protein, 448 aa, Phaeodactylum tricornutum
  misc_feature: cpSRP54
MSEASIQPALREVRRALLDADVNVDVADTLIEGVRARSLGQEVLEGVTAEQQFVKAMYDELLDMMGGDSSVPMSDGPSNVPVATLASGTAADPAVILLAGLQGAGKTTAAGKLALFLKEQRKVLLVAADIYRPAAIKQLQVLGESIGVEVFTKGTDVDPVEIVNAGIQKARDEGYDTVIVDTAGRQVIDTDLMDELQRMKRAASPQETLLIVDAMTGQEAASLTAAFDSAIGLTGAILTKMDGDSRGGAAVSVRGVSGKPIKFVGTGEKTADLEPFYPDRMASRILGMGDVVSLVEKAASEVSDADALKMQQKMLDASFDFDDFVKQSELVTKMGSVAGIAKLMPGMANQLNMNQIREVEARLKKSKSMISSMTKKERANPELLIKDSSARSRLIRITKGSGCGLDEGQQFMSEFQRMKTMMSTRRFWRFWLMIQSLALAVTRPENTV

SEQ ID NO: 11 - protein, 536 aa, Nannochloropsis gaditana
  misc_feature: cpSRP54
MTTISTQSSGRSKGVAYAMMDGITNGLIGALKSLAGQKTISEANIDGALRDVKRALLDADVNLKVTNALLEAVKEKALGMDVTKGVTPDQEFVKIMYDELVDLMGAEQAELAQASKPPTVILLAGLQGAGKTTAAAKLALYCQSRAEKAEAFEKILMVAADVYRPAAIDQLRTLGERIDVEVFSMGTDEDPIVIARKALEKAKAQGFTTVIVDTAGRQVIDEKLMKEIKGVKTAVKPDEVLLVVDAMTGQEAATVTARFNDEIGLTGAILTKLDGDTRGGAALSVRGVSGKPIKFIGVGETLEKLEPFYPDRMASRILGMGDVVSLVEKAQDEINQDDAMAIFKKMMTGTFDFDDFMTQTRMISKMGSLSGMMKMIPGMAGVLPGDAMYEGEKKLFAYQEMINVMEPEERKDPKMLLDNPGADLRWKRIVEESGRSMEEAKNFQREFSNLRLMMTRMSSRLSEKTGFDPSKGKDAAIDESALQELDMKNLAMMSQNRQARRKLEKQSRRAGSDDDTPQKGFGGGGGGGGGKKKKKR

SEQ ID NO: 12 - protein, 486 aa, Thalassiosira pseudonana
  misc_feature: cpSRP54
MFDQLSNALTEVAKNFGGKQRMTENSIQPALKSVRRALLDADVNLDVATALIDGVKRRSLGKEVTKGVTAEQQFIKAMYDELLDMMGGEANESNTMATLAHSSVANEPAVILLAGLQGAGKTTAAGKLAFRLPKRNRKVLLVAADVYRPAAIEQLQILGKQIGVEVFSMGVDADPADIAKEAVEKAKREGFDTVVVDTAGRQVVDEELMEELRRVKKTVEPDETLLVVDAMTGQAAASLTASFDAAVGISGAILTKLDGDSRGGAAVSIRGVSGKPIKFVGVGEKTNDLEPFYPDRMASRILGMGDVISLVEKASMEVSDADAAKMQEKMAKAEFDFDDFMTQSRMVSKMGSMAGVAKMLPGMGNMIDSSQMRQVEERIKRSEAMICSMNKKERANPGLLLTDKSARSRLMRITKGSGLAFEDGLAFMSEFQKMRTMISRMAKQTGMGQPDGEGEMEPAMAGNRNARRAAKKKGKKGGRGGGMGFA

SEQ ID NO: 13 - protein, 530 aa, Aureococcus anophagefferens
  misc_feature: cpSRP54
MTMARRAATAALVLAAAWAFAPPQTKRATTQLYFFDKLAESITAATDVLSGKSRMTEANTKSALRDVRRSLLDADVAKVVVDGFVENVQASALDGEVAEGVDPGQQFVKIVYDELKRVMGGDDDELLFSDDPEAAAKARAGLAYRDDGAPTVVLLCGLQGAGKTTAAAKLALRLKEEEGKTPMLVAADVYRPAAVEQLQILGEQVGVPVYAEAFEAGAGDAVAIATAGVRAAKERGADVVIVDTAGRQVIEESLMAELRSVRAATKPDETLLVLDAMTGQDAASLAKRFDDACPLTGSVLTKLDGDARGGAALSVRAVSGKPIKFVGVGEKVGDLEPFFPARMASRILGMGDVVSLVEKASKQQSAAEAKAVMERTKQAKFNFDDYLDQARMVSNMGSFGAVAKMMPGMGGIDNDQIAAAEAKIKIQASLINSMTPKERGEPDLIIRDKSALARQKRIAAGSGRSVDQAKQFLSEFQQMRTMMAKMAGQAPPDGADAAAAPDPDALLNRAARRAKKKKGGKRKLKTAGFG

SEQ ID NO: 14 - protein, 556 aa, Ectocarpus siliculosus
  misc_feature: cpSRP54
MIMASLKHRSPPRGGAAATLSFFCCVCALFAQSSVAFVPAGGLSRCGVNDRSSSSCRAAAIGAAGRSSLPVSRSSSRRGRRGGCAGGASSPLGMMFDTLAENMAGVANLFTGQKTITESSVEGALNEVKRALLDADLNLMVTNTLVDAVKSKAVGMKLVDGVTAKQQFVNVMNDELVEIMGAEQAPLARRTDGKPTVILLAGLQGTGKTTAAAKLAKYLQQEEEPKKVLLVAGDVYRPAIDQLISLGKRIDVEVFSMGQGVDPVEITKAGLERAVEGEFDTVIVDTAGRQVVDDTLMTELKDIQVASEADEVLLVVDAMTGQEAATLASVFNEKIGITGAVLTKMDGDTRGGAALSVQGVSQKPIKFVGIGEKMSEEEAAKLAKKMINAEFDFNDFLKQAKMMKGMGSLGGVANMIPGMAGKITPQQLNQAEEGVQRAEGLIKFMTPEERRTPKLLILDPTSQARCRRIARDAGVKLSAVSAFLKEFQAMQSNMSRMGKQMADGDPNAGPGGQPSPFQGLGGDTAPGAAPSMNRQQRRQSKKNKAGRSAAPSKGFG

SEQ ID NO: 15 - protein, 196 aa, Parachlorella sp.
  misc_feature: GTPase domain of SEQ ID NO:2
PQVILMAGLQGTGKTTAAGKLALFLQKKGQKVLLVATDIYRPAAIDQLVKLGDRIGVPVFQLGTQVQPPEIARQGLEKARAEGFDAVIVDTAGRLQIDQSMMEELVQIKSTVKPSDTLLVVDAMTGQEAAGLVKAFNDAVDITGAVLTKLDGDSRGGAALSVRQVSGRPIKFVGMGEGMEALEPFYPERMASRILG

SEQ ID NO: 16 - protein, 191 aa, Chlamydomonas reinhardtii
  misc_feature: GTPase domain of SEQ ID NO:3
VHGARGVGKTTAAGKLALYLKKAKKSCLLVATDVYRPAAIDQLVKLGAAIDVPVFEMGTDVSPVEIAKKGVEEARRLGVDAVIIDTAGRLQVDEGMMAELRDVKSAVRPSDTLLVVDAMTGQEAANLVRSFNEAVDISGAILTKMDGDSRGGAALSVREVSGKPIKFVGVGEKMEALEPFYPERMASRILG

SEQ ID NO: 17 - protein, 196 aa, Micromonas pusilla
  misc_feature: GTPase domain of SEQ ID NO:4
PTVILMAGLQGVGKTTACGKLALFLKAQGKQSLLVATDVYRPAAIDQLKKLGEQIDVPVFELGTDFSPPDIARSGVEKAKLENFDVVIVDTAGRLQVDEMLMAELLATKAATRADETLLVVDAMTGQEAASLTAAFNDAVGITGAVLTKMDGDTRGGAALSVREVSGKPIKFIGSGEKLDALEPFFPERMTTRILG

SEQ ID NO: 18 - protein, 196 aa, Micromonas sp.
  misc_feature: GTPase domain of SEQ ID NO:5
PTVILMAGLQGVGKTTACGKLALYLKKQGKDSLLVATDVYRPAAIEQLKRLGEQVKTPVFDMGVRVDPPEVARLGLEKARAEGIDVVIIDTAGRLQVDVHLMEELRATKIATAADEILLVVDAMTGQEAAALTAAFDEAVGITGAVLTKMDGDTRGGAALSVREVSGKPIKFTGVGEKMEALEPFYPERMASRILG

SEQ ID NO: 19 - protein, 195 aa, Paulinella chromatophora
  misc_feature: GTPase domain of SEQ ID NO:6
TVVLMAGLQGAGKTTAAAKLALYLKNQGEKVLMVAADVYRPAAIDQLFVLGKQIDVEVFTLNPESIPEDIAAAGLQKAIREGFDYLIVDTAGRLQIDTAMMQEMVRIRSAVNPNEILLVVDSMIGQEAAELTRAFHEQIGITGAVLTKLDGDARGGAALSIRKVSGAPIKFIGTGEKVEALQPFHPERMASRILG

SEQ ID NO: 20 - protein, 196 aa, Ostreococcus lucimarinus
  misc_feature: GTPase domain of SEQ ID NO:7
PTVVLMAGLQGVGKTTACGKLSLALRKQGKSVLLVATDVYRPAAIDQLKTLGKQIGVPVFDMGVDGNPPEIAARGVRKAKDEDIDVVIVDTAGRLNIDEKLMGELKATKEATSADETLLVVDAMTGQEAATLTASFNEAVEITGAILTKMDGDTRGGAALSVREVSGKPIKFTGVGEKMDALEPFYPERMTSRILG

SEQ ID NO: 21 - protein, 186 aa, Ostreococcus tauri
  misc_feature: GTPase domain of SEQ ID NO:8
PTVILMAGLQGVGKTTACGKLSLAMRKQGKTVLLVATDVYRPAAIDQLKTLGTQIGVPVFDMGVDASPPEVAARGVRKAKEEDIDVVIVDTAGRLNIDEKLMSELKDTKLATKADETLLVVDAMTGQEAANLTASFQRGDGRRTRRGGAALSVARSFRKAHQFTASVKMDALEPFYPERMTSRILG

SEQ ID NO: 22 - protein, 97 aa, Volvox carteri
  misc_feature: GTPase domain of SEQ ID NO:9
PQIILMAGLQGVGKTTAAGKLALYLKKAKKSCLLVATDVYRPAAIDQLVKLGAAIDVPVFELGTQVSGKPIKFVGVGEKMEALEPFYPERMASRILG

SEQ ID NO: 23 - protein, 195 aa, Phaeodactylum tricornutum
  misc_feature: GTPase domain of SEQ ID NO:10
PAVILLAGLQGAGKTTAAGKLALFLKEQRKVLLVAADIYRPAAIKQLQVLGESIGVEVFTKGTDVDPVEIVNAGIQKARDEGYDTVIVDTAGRQVIDTDLMDELQRMKRAASPQETLLIVDAMTGQEAASLTAAFDSAIGLTGAILTKMDGDSRGGAAVSVRGVSGKPIKFVGTGEKTADLEPFYPDRMASRILG

SEQ ID NO: 24 - protein, 202 aa, Nannochloropsis gaditana
  misc_feature: GTPase domain of SEQ ID NO:11
PTVILLAGLQGAGKTTAAAKLALYCQSRAEKAEAFEKILMVAADVYRPAAIDQLRTLGERIDVEVFSMGTDEDPIVIARKALEKAKAQGFTTVIVDTAGRQVIDEKLMKEIKGVKTAVKPDEVLLVVDAMTGQEAATVTARFNDEIGLTGAILTKLDGDTRGGAALSVRGVSGKPIKFIGVGETLEKLEPFYPDRMASRILG

SEQ ID NO: 25 - protein, 196 aa, Thalassiosira pseudonana
  misc_feature: GTPase domain of SEQ ID NO:12
PAVILLAGLQGAGKTTAAGKLAFRLPKRNRKVLLVAADVYRPAAIEQLQILGKQIGVEVFSMGVDADPADIAKEAVEKAKREGFDTVVVDTAGRQVVDEELMEELRRVKKTVEPDETLLVVDAMTGQAAASLTASFDAAVGISGAILTKLDGDSRGGAAVSIRGVSGKPIKFVGVGEKTNDLEPFYPDRMASRILG

SEQ ID NO: 26 - protein, 200 aa, Aureococcus anophagefferens
  misc_feature: GTPase domain of SEQ ID NO:13
PTVVLLCGLQGAGKTTAAAKLALRLKEEEGKTPMLVAADVYRPAAVEQLQILGEQVGVPVYAEAFEAGAGDAVAIATAGVRAAKERGADVVIVDTAGRQVIEESLMAELRSVRAATKPDETLLVLDAMTGQDAASLAKRFDDACPLTGSVLTKLDGDARGGAALSVRAVSGKPIKFVGVGEKVGDLEPFFPARMASRILG

SEQ ID NO: 27 - protein, 185 aa, Ectocarpus siliculosus
  misc_feature: GTPase domain of SEQ ID NO:14
PTVILLAGLQGTGKTTAAAKLAKYLQQEEEPKKVLLVAGDVYRPAIDQLISLGKRIDVEVFSMGQGVDPVEITKAGLERAVEGEFDTVIVDTAGRQVVDDTLMTELKDIQVASEADEVLLVVDAMTGQEAATLASVFNEKIGITGAVLTKMDGDTRGGAALSVQGVSQKPIKFVGIGEKMSEEEA

SEQ ID NO: 28 - DNA, 1611 bp, Nannochloropsis gaditana
  misc_feature: cpSRP54
atgacaaccatttcgacgcaaagctcaggacggagcaagggcgtggcctacgccatgatggacggcattaccaatggtctcatcggggctttgaagtctttggcagggcaaaaaaccatctcagaagccaatatcgacggcgccctgcgcgacgtcaagcgggccctgctagacgcggacgtgaaccttaaggtgactaacgccttgctggaggcggttaaagagaaggcactcggcatggacgtgaccaaaggcgtgacccccgaccaggagttcgtcaagatcatgtacgacgagctcgtcgacctgatgggcgccgagcaggcggaactcgcgcaggccagcaagccccccactgtcatcctcctggctgggctgcagggtgccggtaaaaccacggctgccgccaagcttgccctctactgccagtcccgcgccgagaaagccgaggcctttgaaaagatattgatggtggcggcggacgtgtaccgcccggcagccatcgaccagctccgtacgctgggagaaaggattgacgtggaggttttctccatgggcactgacgaggacccgatagtcatcgcccgcaaggccctggagaaggcgaaagcccagggctttaccaccgtcattgtcgacaccgcgggcaggcaggtcatcgacgagaagctgatgaaggagatcaagggggtcaaaaccgccgtcaagcccgacgaagtcctcctggtcgtggacgccatgacgggccaagaggccgccaccgtcaccgcccgcttcaacgacgaaatcggacttaccggggctatcctgaccaagctggacggtgacacgcgcggtggagccgccctctctgtccgaggtgtgagtgggaagcccatcaaattcatcggagtcggtgaaacgctggaaaaactcgaaccgttctaccccgaccgcatggccagtcggatcctgggcatgggcgacgtggtgtccctggtggagaaagcacaagatgagatcaaccaggacgacgccatggccatcttcaaaaagatgatgaccggcaccttcgatttcgatgacttcatgacccagacccgcatgatttccaagatgggcagcctctcaggcatgatgaagatgatcccgggcatggccggcgtccttcccggcgacgccatgtacgagggcgagaagaagctcttcgcctaccaggaaatgatcaacgtgatggagccggaggagcggaaagacccgaagatgcttctggacaaccccggcgcggacctacgatggaagcgcatcgtggaagagagcggtcggtccatggaggaggcgaagaacttccagcgagagttttcgaacctgcgtttgatgatgacgcgtatgtcaagccgactcagcgagaagacaggctttgaccccagcaagggcaaggacgccgccattgacgagtcggcgctgcaggagctagacatgaagaatctggcgatgatgagtcagaacaggcaagcgcggcgaaagctggaaaaacaatctcgtcgagcaggaagtgatgatgacacaccgcaaaaaggctttggaggaggaggtggtgggggaggaggcaagaagaagaaaaagcgatga

SEQ ID NO: 29 - DNA, 1689 bp, Nannochloropsis gaditana
  misc_feature: cytoSRP54
atggtgttgcaggagctcggtgacaagcttacgggggctctacgccggctgcagaccaccacggtcgtcaacgacgacgtcctcaacgacctgctccaggacgtatgccgtgcgttagtcgaatccgatgtgaatatcaaggtagtggcgaccctaagaaagggcatcaaggagaaagtcaaccttgcagatgcccccgctggcctgaacagacggaaaatggtgcagcgggcggtgatggaggaattggtccgcctggtcgactcgggaacaaagccgtaccaaatgaggaagggaaagtcgaacgtgatcatgtttgtgggcttgcaaggctcggggaaaactaccaccattgccaaatacgccaactattaccagcggaagggatggaagacgtgcatggtgtgtgccgatacctttcgtgccggagccttcgatcagctgaagcagaatgcgacaaaactccgtgtgcctttttacggctcctacacggaggcggacccggtacggatcgccgaggagggcgtccagcagttccgttcagagggatacgaggttatcattgtcgatacctcgggccggcacaagcaggaagaagccctgtttgaggagatgaaagagatccaagcggcggtccgtcccgacaacgtggtgtacgtcatggacgccacccagggccaagccgtcttcgaccaggcacagggtttccaccaggccgccgcggtgggctccgtcattgtcaccaagctggacgggcacgccaaggggggaggcgccttgtcggccgtggcggcgacgggggcgcctatcatatttttgggctcgggggagcattttgacgacctggacgtcttcaaccccgggagtttcatcagtcggttgctgggcttgggggacatgcggggttttttggaggaagtgagcagcctgggggcgagggaaggagggaaagagaggcaggaggccatggcccagcggctcgtcaagggccagttcaccctccgcgacatgtacgagcagtttgagaacgtgatgaagctggggcccctttccaaggtcatgggcatgctgccgggctttccctcttttctgatgggggggggggaaggagggaggggggggcaggacgaagctgccacgggccggctgaagcgtttcttgaccatgatggacagcatgacggacgcggagctcgatgggaaggtggacctgaacaagagcgagagccgcgtgaaccggattgctcgaggaagcggggcacacccgatggaagtccaatttttgctcaagacgtacgcgcaattctcgcaaatgttcaagaagatgggcccgatgatgttgaaaggcggggagggtggcatacagcggcagatggcacgcaacccgggaggcgtgatgaatcagttgagcaaggcggtggacccgcgaatgctacagcagatgggaggcgcaaaaggaatgatggacatgatgaaagcgatgggaggaggaatggggggggggcttgcggacatgctgcagaacttggggggaggggggggagggagagggggaggaagagggagtggacgaggagggggtgggatggatccagaacagatgcaggcgcagatggcgcaaatggaagagatgatgaaaagtatgggaatgggtggaggagggaaaggaggtggagggttccctttctga

SEQ ID NO: 30 - protein, 562 aa, Nannochloropsis gaditana
  misc_feature: cytoSRP54
MVLQELGDKLTGALRRLQTTTVVNDDVLNDLLQDVCRALVESDVNIKVVATLRKGIKEKVNLADAPAGLNRRKMVQRAVMEELVRLVDSGTKPYQMRKGKSNVIMFVGLQGSGKTTTIAKYANYYQRKGWKTCMVCADTFRAGAFDQLKQNATKLRVPFYGSYTEADPVRIAEEGVQQFRSEGYEVIIVDTSGRHKQEEALFEEMKEIQAAVRPDNVVYVMDATQGQAVFDQAQGFHQAAAVGSVIVTKLDGHAKGGGALSAVAATGAPIIFLGSGEHFDDLDVFNPGSFISRLLGLGDMRGFLEEVSSLGAREGGKERQEAMAQRLVKGQFTLRDMYEQFENVMKLGPLSKVMGMLPGFPSFLMGGGEGGRGGQDEAATGRLKRFLTMMDSMTDAELDGKVDLNKSESRVNRIARGSGAHPMEVQFLLKTYAQFSQMFKKMGPMMLKGGEGGIQRQMARNPGGVMNQLSKAVDPRMLQQMGGAKGMMDMMKAMGGGMGGGLADMLQNLGGGGGGRGGGRGSGRGGGGMDPEQMQAQMAQMEEMMKSMGMGGGGKGGGGFPF

SEQ ID NO: 31 - DNA, 11263 bp, Artificial Sequence
  Unknown
  misc_feature: Construct pSGE-6206 for expressing Cas9
gcggccgccgtatggtcgacggttgctcggatggggggggcggggagcgatggagggaggaagatcaggtaaggtctcgacagactagagaagcacgagtgcaggtataagaaacagcaaaaaaaagtaatgggcccaggcctggagagggtatttgtcttgtttttctttggccaggaacttgttctcctttcttcgtttctaggaccccgatccccgctcgcatttctctcttcctcagccgaagcgcagcggtaaagcatccattttatcccaccgaaagggcgctcccagccttcgtcgagcggaaccggggttacagtgcctcaaccctcccagacgtagccagagggaagcaactccctgatgccaaccgctgtgggctgcccatcggaatctttgacaattgccttgatccccgggtgcaagtcaagcagcacctgccgacatcgcccgcacggagacagaatgccgcggttttcgttcccgatggccactatgcacgtcagatttccggcagcagccgcagcggccgttccgaggaccacgagctccgcgcatggccctccggtgaaatgatatacattcacgccggtaaagatccgaccgtcggacgagagggctgcactggccaccgagtagtcctcgctaataggtatgctgttgatggtcgcagttgcacgttcgatcagcgtggattcctcttgggataaaggcttggccatcgagctcggtacccggggatccatgattgttgtattatgtacctatgtttgtgatgagacaataaatatgagaagagaacgttgcggccacttttttctccttccttcgcgtgctcatgttggtggtttgggaggcagaagatgcatggagcgccacacattcggtaggacgaaacagcctcccccacaaagggaccatgggtagctaggatgacgcacaagcgagttcccgctctcgaagggaaacccaggcatttccttcctcttttcaagccacttgttcacgtgtcaacacaattttggactaaaatgcccctcggaactcggcaggcctccctctgctccgttgtcctggtcgccgagaacgcgagaccgtgccgcatgccatcgatctgctcgtctgtactactaatcgtgtgcgtgttcgtgcttgtttcgcacgaaattgtcctcgttcggccctcacaacggtggaaatcggtgctagaataaagtgaggtggcttatttcaatggcggccgtcatcatgcgggatcaactgaagtacggcgggttctcgagatttcatcgtgctcgtccagagcaggtgttttgcctgcagctcttcatgtttaggggtcatgatttcatctgatatgccgtaagaaaaccaatattcacttctcaattttccatggaaaggtgaaggcctaggttgtgtgcgaggcaacgactggggagggatcgcaacattcttgctaacctcccctctatcttggccgctgtgaatcggcatatttaccgggctgaattgagaaagtgttttgagggaattaaaaggtggctgtcttgcaagcttggcttcagtgcctgcttaattcgaaccgatccagcttgtgatgaggccttcctaagcctggtagtcagaagcgacatggcgctataaatttcgtctcagttggagagtagaaaagcatgattcgaacacggttttcaactgccaaagatatctccattgtttccttcaatctgtacacctgcacggtgcaccagttggtacggcatattatggtttaataagcatacatcatatgaatacaattcagcttaaatttatcatacaaagatgtaagtgcagcgtgggtctgtaacgatcgggcgtaatttaagataatgcgagggaccgggggaggttttggaacggaatgaggaatgggtcatggcccataataataatatgggtttggtcgcctcgcacagcaaccgtacgtgcgaaaaaggaacagatccatttaataagttgaacgttattctttcctatgcaatgcgtgtatcggaggcgagagcaagtcataggtggctgcgcacaataattgagtctcagctgagcgccgtccgcgggtggtgtgagtggtcatcctcctcccggcctatcgctcacatcgcctctcaatggtggtggtggggcctgatatgacctcaatgccgacccatattaaaacccagtaaagcattcaccaacgaacgaggggctcttttgtgtgtgttttgagtatgattttacacctctttgtgcatctctctggtcttccttggttcccgtagtttgggcatcatcactcacgcttccctcgaccttcgttcttcctttacaaccccgacacaggtcagagttggagtaatcaaaaaaggggtgcacgaatgagatacattagattttgacagatatccttttactggagagggttcaagggatcaaatgaacagcgggcgttggcaatctagggagggatcggaggttggcagcgagcgaaagcgtgtccatccttttggctgtcacacctcacgaaccaactgttagcaggccagcacagatgacatacgagaatctttattatatcgtagaccttatgtggatgacctttggtgctgtgtgtctggcaatgaacctgaaggcttgatagggaggtggctcccgtaaaccctttgtcctttccacgctgagtctcccccgcactgtcctttatacaaattgttacagtcatctgcaggcggtttttctttggcaggcaaagatgcccaagaaaaagcggaaggtcggcgactacaaggatgacgatgacaagttggagcctggagagaagccctacaaatgccctgagtgcggaaagagcttcagccaatctggagccttgacccggcatcaacgaacgcatacacgagacaagaagtactccatcgggctggacatcgggacgaactccgtgggatgggccgtgatcacagacgaatacaaggtgccttccaagaagttcaaggtgctggggaacacggacagacactccatcaagaagaacctcatcggggccttgctcttcgactccggagaaaccgccgaagcaacgcgattgaaaagaaccgccagaagacgatacacacgacggaagaaccgcatctgctacctccaggagatcttcagcaacgagatggccaaggtggacgactcgttctttcatcgcctggaggagagcttcctggtggaggaagacaagaaacatgagcgccacccgatcttcgggaacatcgtggacgaagtggcctaccacgagaaataccccacgatctaccacttgcgcaagaaactcgtggactccacggacaaagcggacttgcggttgatctacttggccttggcccacatgatcaaatttcggggccacttcctgatcgagggcgacttgaatcccgacaattccgacgtggacaagctcttcatccagctggtgcagacctacaaccagctcttcgaggagaaccccatcaatgcctccggagtggacgccaaagccatcttgtccgcccgattgtccaaatccagacgcttggagaacttgatcgcacaacttcctggcgagaagaagaacggcctcttcggcaacttgatcgcgctgtcgctgggattgacgcctaacttcaagtccaacttcgacttggccgaggacgccaagttgcaactgtccaaggacacctacgacgacgacctcgacaacctgctggcccaaattggcgaccaatacgcggacttgtttttggcggccaagaacttgagcgacgccatcttgttgagcgacatcttgcgcgtgaatacggagatcaccaaagcccctttgtccgcctctatgatcaagcggtacgacgagcaccaccaagacttgaccctgttgaaagccctcgtgcggcaacaattgcccgagaagtacaaggagatcttcttcgaccagtccaagaacgggtacgccggctacatcgacggaggagcctcccaagaagagttctacaagttcatcaagcccatcctggagaagatggacggcaccgaggagttgctcgtgaagctgaaccgcgaagacttgttgcgaaaacagcggacgttcgacaatggcagcatcccccaccaaatccatttgggagagttgcacgccatcttgcgacggcaagaggacttctacccgttcctgaaggacaaccgcgagaaaatcgagaagatcctgacgttcagaatcccctactacgtgggacccttggcccgaggcaattcccggtttgcatggatgacgcgcaaaagcgaagagacgatcaccccctggaacttcgaagaagtggtcgacaaaggagcatccgcacagagcttcatcgagcgaatgacgaacttcgacaagaacctgcccaacgagaaggtgttgcccaagcattcgctgctgtacgagtacttcacggtgtacaacgagctgaccaaggtgaagtacgtgaccgagggcatgcgcaaacccgcgttcctgtcgggagagcaaaagaaggccattgtggacctgctgttcaagaccaaccggaaggtgaccgtgaaacagctgaaagaggactacttcaagaagatcgagtgcttcgactccgtggagatctccggcgtggaggaccgattcaatgcctccttgggaacctaccatgacctcctgaagatcatcaaggacaaggacttcctggacaacgaggagaacgaggacatcctggaggacatcgtgctgaccctgaccctgttcgaggaccgagagatgatcgaggaacggttgaaaacgtacgcccacttgttcgacgacaaggtgatgaagcagctgaaacgccgccgctacaccggatggggacgattgagccgcaaactgattaatggaattcgcgacaagcaatccggaaagaccatcctggacttcctgaagtccgacgggttcgccaaccgcaacttcatgcagctcatccacgacgactccttgaccttcaaggaggacatccagaaggcccaagtgtccggacaaggagactccttgcacgagcacatcgccaatttggccggatcccccgcaatcaaaaaaggcatcttgcaaaccgtgaaagtggtcgacgaactggtgaaggtgatgggacggcacaagcccgagaacatcgtgatcgaaatggcccgcgagaaccaaaccacccaaaaaggacagaagaactcccgagagcgcatgaagcggatcgaagagggcatcaaggagttgggctcccagatcctgaaggagcatcccgtggagaatacccaattgcaaaacgagaagctctacctctactacctccagaacgggcgggacatgtacgtcgaccaagagctggacatcaaccgcctctccgactacgatgtggatcatattgtgccccagagcttcctcaaggacgacagcatcgacaacaaggtcctgacgcgcagcgacaagaaccggggcaagtctgacaatgtgccttccgaagaagtcgtgaagaagatgaagaactactggcggcagctgctcaacgccaagctcatcacccaacggaagttcgacaacctgaccaaggccgagagaggaggattgtccgagttggacaaagccggcttcattaaacgccaactcgtggagacccgccagatcacgaagcacgtggcccaaatcttggactcccggatgaacacgaaatacgacgagaatgacaagctgatccgcgaggtgaaggtgatcacgctgaagtccaagctggtgagcgacttccggaaggacttccagttctacaaggtgcgggagatcaacaactaccatcacgcccatgacgcctacctgaacgccgtggtcggaaccgccctgatcaagaaataccccaagctggagtccgaattcgtgtacggagattacaaggtctacgacgtgcggaagatgatcgcgaagtccgagcaggagatcggcaaagccaccgccaagtacttcttttactccaacatcatgaacttcttcaagaccgagatcacgctcgccaacggcgagatccgcaagcgccccctgatcgagaccaacggcgagacgggagagattgtgtgggacaaaggaagagattttgccacagtgcgcaaggtgctgtccatgcctcaggtgaacatcgtgaagaagaccgaggtgcaaacaggagggttttccaaagagtccattttgcctaagaggaattccgacaagctcatcgcccgcaagaaggactgggaccccaagaagtacgggggcttcgactcccccacggtggcctactccgtgttggtggtggccaaagtggagaaagggaagagcaagaagctgaaatccgtgaaggagttgctcggaatcacgatcatggaacgatcgtcgttcgagaaaaaccccatcgacttcctcgaagccaaagggtacaaagaggtgaagaaggacctgatcatcaagctgcccaagtactccctgttcgagctggagaacggccgcaagcggatgctggcctccgccggggaactgcagaaagggaacgaattggccttgccctccaaatacgtgaacttcctctacttggcctcccattacgaaaagctcaaaggatcccctgaggacaatgagcagaagcaactcttcgtggaacaacacaagcactacctggacgagatcatcgagcagatcagcgagttctccaagcgcgtgatcctcgccgacgccaacctggacaaggtgctctccgcctacaacaagcaccgcgacaagcctatccgcgagcaagccgagaatatcattcacctgtttaccctgacgaatttgggagcccctgccgcctttaaatactttgacaccaccatcgaccgcaaaagatacacctccaccaaggaagtcttggacgccaccctcatccaccagtccatcacgggcctctacgagacgcgcatcgacctctcccaattgggcggcgactaaagtgatgcggcctttaggaaacaccacaaaagtaattgacaatctcaggaacgatctgcgtgtttacagcttcccaaataacaattataccacgtaccaaaaggggtttaatgtatctcacaaattcttctaataggtacagcttctcaaattgggtgtatgatgtgacacttcgtctcacacacgtcacgataattcagcgtatggcttcccttcatcacattcacgcaaacttctacacaaccctgggcatatttcttgtgttggcaacactcccgaaatcgattctgcacacaatggttcattcaatgattcaagtacgttttagacggactaggcagtttaattaaaaacatctatcctccagatcaccagggccagtgaggccggcataaaggacggcaaggaaagaaaagaaagaaagaaaaggacacttatagcatagtttgaagttataagtagtcgcaatctgtgtgcagccgacagatgctttttttttccgtttggcaggaggtgtagggatgtcgaagaccagtccagctagtatctatcctacaagtcaatcatgctgcgacaaaaatttctcgcacgaggcctctcgataaacaaaactttaaaagcacacttcattgtcatgcagagtaataactcttccgcgtcgatcaatttatcaatctctatcatttccgcccctttccttgcatagagcaagaaaagcgacccggatgaggataacatgtcctgcgccagtagtgtggcattgcctgtctctcatttacacgtactgaaagcataatgcacgcgcataccaatatttttcgtgtacggagatgaagagacgcgacacgtaagatcacgagaaggcgagcacggttgccaatggcagacgcgctagtctccattatcgcgttgttcggtagcttgctgcatgtcttcagtggcactatatccactctgcctcgtcttctacacgagggccacatcggtgcaagttcgaaaaatcatatctcaatcttcagatcctttccagaaacggtgctcaggcgggaaagtgaaggttttctactctagtggctaccccaattctctccgactgtcgcagacggtccttcgttgcgcacgcaccgcgcactacctctgaaattcgacaaccgaagttcaattttacatctaacttctttcccattctctcaccaaaagcctagcttacatgttggagagcgacgagagcggcctgcccgccatggagatcgagtgccgcatcaccggcaccctgaacggcgtggagttcgagctggtgggcggcggagagggcacccccgagcagggccgcatgaccaacaagatgaagagcaccaaaggcgccctgaccttcagcccctacctgctgagccacgtgatgggctacggcttctaccacttcggcacctaccccagcggctacgagaaccccttcctgcacgccatcaacaacggcggctacaccaacacccgcatcgagaagtacgaggacggcggcgtgctgcacgtgagcttcagctaccgctacgaggccggccgcgtgatcggcgacttcaaggtgatgggcaccggcttccccgaggacagcgtgatcttcaccgacaagatcatccgcagcaacgccaccgtggagcacctgcaccccatgggcgataacgatctggatggcagcttcacccgcaccttcagcctgcgcgacggcggctactacagctccgtggtggacagccacatgcacttcaagagcgccatccaccccagcatcctgcagaacgggggccccatgttcgccttccgccgcgtggaggaggatcacagcaacaccgagctgggcatcgtggagtaccagcacgccttcaagaccccggatgcagatgccggtgaagaataagggtgggaaggagtcggggagggtcctggcagagcggcgtcctcatgatgtgttggagacctggagagtcgagagcttcctcgtcacctgattgtcatgtgtgtataggttaagggggcccactcaaagccataaagacgaacacaaacactaatctcaacaaagtctactagcatgccgtctgtccatctttatttcctggcgcgcctatgcttgtaaaccgttttgtgaaaaaatttttaaaataaaaaaggggacctctagggtccccaattaattagtaatataatctattaaaggtcattcaaaaggtcatccagacgaaagggcctcgtgatacgcctatttttataggttaatgtcatgataataatggtttcttagacgtcaggtggcacttttcggggaaatgtgcgcggaacccctatttgtttatttttctaaatacattcaaatatgtatccgctcatgagacaataaccctgataaatgcttcaataatattgaaaaaggaagagtatgagtattcaacatttccgtgtcgcccttattcccttttttgcggcattttgccttcctgtttttgctcacccagaaacgctggtgaaagtaaaagatgctgaagatcagttgggtgcacgagtgggttacatcgaactggatctcaacagcggtaagatccttgagagttttcgccccgaagaacgttttccaatgatgagcacttttaaagttctgctatgtggcgcggtattatcccgtattgacgccgggcaagagcaactcggtcgccgcatacactattctcagaatgacttggttgagtactcaccagtcacagaaaagcatcttacggatggcatgacagtaagagaattatgcagtgctgccataaccatgagtgataacactgcggccaacttacttctgacaacgatcggaggaccgaaggagctaaccgcttttttgcacaacatgggggatcatgtaactcgccttgatcgttgggaaccggagctgaatgaagccataccaaacgacgagcgtgacaccacgatgcctgtagcaatggcaacaacgttgcgcaaactattaactggcgaactacttactctagcttcccggcaacaattaatagactggatggaggcggataaagttgcaggaccacttctgcgctcggcccttccggctggctggtttattgctgataaatctggagccggtgagcgtgggtctcgcggtatcattgcagcactggggccagatggtaagccctcccgtatcgtagttatctacacgacggggagtcaggcaactatggatgaacgaaatagacagatcgctgagataggtgcctcactgattaagcattggtaactgtcagaccaagtttactcatatatactttagattgatttaaaacttcatttttaatttaaaaggatctaggtgaagatcctttttgataatctcatgaccaaaatcccttaacgtgagttttcgttccactgagcgtcagaccccgtagaaaagatcaaaggatcttcttgagatcctttttttctgcgcgtaatctgctgcttgcaaacaaaaaaaccaccgctaccagcggtggtttgtttgccggatcaagagctaccaactctttttccgaaggtaactggcttcagcagagcgcagataccaaatactgtccttctagtgtagccgtagttaggccaccacttcaagaactctgtagcaccgcctacatacctcgctctgctaatcctgttaccagtggctgctgccagtggcgataagtcgtgtcttaccgggttggactcaagacgatagttaccggataaggcgcagcggtcgggctgaacggggggttcgtgcacacagcccagcttggagcgaacgacctacaccgaactgagatacctacagcgtgagctatgagaaagcgccacgcttcccgaagggagaaaggcggacaggtatccggtaagcggcagggtcggaacaggagagcgcacgagggagcttccagggggaaacgcctggtatctttatagtcctgtcgggtttcgccacctctgacttgagcgtcgatttttgtgatgctcgtcaggggggcggagcctatggaaaaacgccagcaacgcggcctttttacggttcctggccttttgctggccttttgctcacatgttctttcctgcgttatcccctgattctgtggataaccgtattaccgcctttgagtgagctgataccgctcgccgcagccgaacgaccgagcgcagcgagtcagtgagcgaggaagcggaaga

SEQ ID NO: 32 - DNA, 4101 bp, Artificial Sequence
  Unknown
  misc_feature: Cas9 gene codon-optimized for Nannochloropsis
gacaagaagtactccatcgggctggacatcgggacgaactccgtgggatgggccgtgatcacagacgaatacaaggtgccttccaagaagttcaaggtgctggggaacacggacagacactccatcaagaagaacctcatcggggccttgctcttcgactccggagaaaccgccgaagcaacgcgattgaaaagaaccgccagaagacgatacacacgacggaagaaccgcatctgctacctccaggagatcttcagcaacgagatggccaaggtggacgactcgttctttcatcgcctggaggagagcttcctggtggaggaagacaagaaacatgagcgccacccgatcttcgggaacatcgtggacgaagtggcctaccacgagaaataccccacgatctaccacttgcgcaagaaactcgtggactccacggacaaagcggacttgcggttgatctacttggccttggcccacatgatcaaatttcggggccacttcctgatcgagggcgacttgaatcccgacaattccgacgtggacaagctcttcatccagctggtgcagacctacaaccagctcttcgaggagaaccccatcaatgcctccggagtggacgccaaagccatcttgtccgcccgattgtccaaatccagacgcttggagaacttgatcgcacaacttcctggcgagaagaagaacggcctcttcggcaacttgatcgcgctgtcgctgggattgacgcctaacttcaagtccaacttcgacttggccgaggacgccaagttgcaactgtccaaggacacctacgacgacgacctcgacaacctgctggcccaaattggcgaccaatacgcggacttgtttttggcggccaagaacttgagcgacgccatcttgttgagcgacatcttgcgcgtgaatacggagatcaccaaagcccctttgtccgcctctatgatcaagcggtacgacgagcaccaccaagacttgaccctgttgaaagccctcgtgcggcaacaattgcccgagaagtacaaggagatcttcttcgaccagtccaagaacgggtacgccggctacatcgacggaggagcctcccaagaagagttctacaagttcatcaagcccatcctggagaagatggacggcaccgaggagttgctcgtgaagctgaaccgcgaagacttgttgcgaaaacagcggacgttcgacaatggcagcatcccccaccaaatccatttgggagagttgcacgccatcttgcgacggcaagaggacttctacccgttcctgaaggacaaccgcgagaaaatcgagaagatcctgacgttcagaatcccctactacgtgggacccttggcccgaggcaattcccggtttgcatggatgacgcgcaaaagcgaagagacgatcaccccctggaacttcgaagaagtggtcgacaaaggagcatccgcacagagcttcatcgagcgaatgacgaacttcgacaagaacctgcccaacgagaaggtgttgcccaagcattcgctgctgtacgagtacttcacggtgtacaacgagctgaccaaggtgaagtacgtgaccgagggcatgcgcaaacccgcgttcctgtcgggagagcaaaagaaggccattgtggacctgctgttcaagaccaaccggaaggtgaccgtgaaacagctgaaagaggactacttcaagaagatcgagtgcttcgactccgtggagatctccggcgtggaggaccgattcaatgcctccttgggaacctaccatgacctcctgaagatcatcaaggacaaggacttcctggacaacgaggagaacgaggacatcctggaggacatcgtgctgaccctgaccctgttcgaggaccgagagatgatcgaggaacggttgaaaacgtacgcccacttgttcgacgacaaggtgatgaagcagctgaaacgccgccgctacaccggatggggacgattgagccgcaaactgattaatggaattcgcgacaagcaatccggaaagaccatcctggacttcctgaagtccgacgggttcgccaaccgcaacttcatgcagctcatccacgacgactccttgaccttcaaggaggacatccagaaggcccaagtgtccggacaaggagactccttgcacgagcacatcgccaatttggccggatcccccgcaatcaaaaaaggcatcttgcaaaccgtgaaagtggtcgacgaactggtgaaggtgatgggacggcacaagcccgagaacatcgtgatcgaaatggcccgcgagaaccaaaccacccaaaaaggacagaagaactcccgagagcgcatgaagcggatcgaagagggcatcaaggagttgggctcccagatcctgaaggagcatcccgtggagaatacccaattgcaaaacgagaagctctacctctactacctccagaacgggcgggacatgtacgtcgaccaagagctggacatcaaccgcctctccgactacgatgtggatcatattgtgccccagagcttcctcaaggacgacagcatcgacaacaaggtcctgacgcgcagcgacaagaaccggggcaagtctgacaatgtgccttccgaagaagtcgtgaagaagatgaagaactactggcggcagctgctcaacgccaagctcatcacccaacggaagttcgacaacctgaccaaggccgagagaggaggattgtccgagttggacaaagccggcttcattaaacgccaactcgtggagacccgccagatcacgaagcacgtggcccaaatcttggactcccggatgaacacgaaatacgacgagaatgacaagctgatccgcgaggtgaaggtgatcacgctgaagtccaagctggtgagcgacttccggaaggacttccagttctacaaggtgcgggagatcaacaactaccatcacgcccatgacgcctacctgaacgccgtggtcggaaccgccctgatcaagaaataccccaagctggagtccgaattcgtgtacggagattacaaggtctacgacgtgcggaagatgatcgcgaagtccgagcaggagatcggcaaagccaccgccaagtacttcttttactccaacatcatgaacttcttcaagaccgagatcacgctcgccaacggcgagatccgcaagcgccccctgatcgagaccaacggcgagacgggagagattgtgtgggacaaaggaagagattttgccacagtgcgcaaggtgctgtccatgcctcaggtgaacatcgtgaagaagaccgaggtgcaaacaggagggttttccaaagagtccattttgcctaagaggaattccgacaagctcatcgcccgcaagaaggactgggaccccaagaagtacgggggcttcgactcccccacggtggcctactccgtgttggtggtggccaaagtggagaaagggaagagcaagaagctgaaatccgtgaaggagttgctcggaatcacgatcatggaacgatcgtcgttcgagaaaaaccccatcgacttcctcgaagccaaagggtacaaagaggtgaagaaggacctgatcatcaagctgcccaagtactccctgttcgagctggagaacggccgcaagcggatgctggcctccgccggggaactgcagaaagggaacgaattggccttgccctccaaatacgtgaacttcctctacttggcctcccattacgaaaagctcaaaggatcccctgaggacaatgagcagaagcaactcttcgtggaacaacacaagcactacctggacgagatcatcgagcagatcagcgagttctccaagcgcgtgatcctcgccgacgccaacctggacaaggtgctctccgcctacaacaagcaccgcgacaagcctatccgcgagcaagccgagaatatcattcacctgtttaccctgacgaatttgggagcccctgccgcctttaaatactttgacaccaccatcgaccgcaaaagatacacctccaccaaggaagtcttggacgccaccctcatccaccagtccatcacgggcctctacgagacgcgcatcgacctctcccaattgggcggcgac

SEQ ID NO: 33 - DNA, 24 bp, Artificial Sequence
  Unknown
  misc_feature: Encodes FLAG tag
gactacaaggatgacgatgacaag

SEQ ID NO: 34 - DNA, 24 bp, Artificial Sequence
  Unknown
  misc_feature: Encodes nuclear localization signal
cccaagaaaaagcggaaggtcggc

SEQ ID NO: 35 - DNA, 147 bp, Artificial Sequence
  Unknown
  misc_feature: Encodes peptide linker
atgcccaagaaaaagcggaaggtcggcgactacaaggatgacgatgacaagttggagcctggagagaagccctacaaatgccctgagtgcggaaagagcttcagccaatctggagccttgacccggcatcaacgaacgcatacacga

SEQ ID NO: 36 - DNA, 1000 bp, Nannochloropsis gaditana
  misc_feature: RPL24 promoter
aataagcatacatcatatgaatacaattcagcttaaatttatcatacaaagatgtaagtgcagcgtgggtctgtaacgatcgggcgtaatttaagataatgcgagggaccgggggaggttttggaacggaatgaggaatgggtcatggcccataataataatatgggtttggtcgcctcgcacagcaaccgtacgtgcgaaaaaggaacagatccatttaataagttgaacgttattctttcctatgcaatgcgtgtatcggaggcgagagcaagtcataggtggctgcgcacaataattgagtctcagctgagcgccgtccgcgggtggtgtgagtggtcatcctcctcccggcctatcgctcacatcgcctctcaatggtggtggtggggcctgatatgacctcaatgccgacccatattaaaacccagtaaagcattcaccaacgaacgaggggctcttttgtgtgtgttttgagtatgattttacacctctttgtgcatctctctggtcttccttggttcccgtagtttgggcatcatcactcacgcttccctcgaccttcgttcttcctttacaaccccgacacaggtcagagttggagtaatcaaaaaaggggtgcacgaatgagatacattagattttgacagatatccttttactggagagggttcaagggatcaaatgaacagcgggcgttggcaatctagggagggatcggaggttggcagcgagcgaaagcgtgtccatccttttggctgtcacacctcacgaaccaactgttagcaggccagcacagatgacatacgagaatctttattatatcgtagaccttatgtggatgacctttggtgctgtgtgtctggcaatgaacctgaaggcttgatagggaggtggctcccgtaaaccctttgtcctttccacgctgagtctcccccgcactgtcctttatacaaattgttacagtcatctgcaggcggtttttctttggcaggcaaag

SEQ ID NO: 37 - DNA, 317 bp, Nannochloropsis gaditana
  misc_feature: Bidirectional terminator 2
agtgatgcggcctttaggaaacaccacaaaagtaattgacaatctcaggaacgatctgcgtgtttacagcttcccaaataacaattataccacgtaccaaaaggggtttaatgtatctcacaaattcttctaataggtacagcttctcaaattgggtgtatgatgtgacacttcgtctcacacacgtcacgataattcagcgtatggcttcccttcatcacattcacgcaaacttctacacaaccctgggcatatttcttgtgttggcaacactcccgaaatcgattctgcacacaatggttcattcaatgattcaa

SEQ ID NO: 38 - DNA, 399 bp, Artificial Sequence
  Unknown
  misc_feature: Aspergillus terreus BLAST gene codon optimized for N. gaditana
atggccaagcctttatcccaagaggaatccacgctgatcgaacgtgcaactgcgaccatcaacagcatacctattagcgaggactactcggtggccagtgcagccctctcgtccgacggtcggatctttaccggcgtgaatgtatatcatttcaccggagggccatgcgcggagctcgtggtcctcggaacggccgctgcggctgctgccggaaatctgacgtgcatagtggccatcgggaacgaaaaccgcggcattctgtctccgtgcgggcgatgtcggcaggtgctgcttgacttgcacccggggatcaaggcaattgtcaaagattccgatgggcagcccacagcggttggcatcagggagttgcttccctctggctacgtctgggagggttga

SEQ ID NO: 39 - DNA, 999 bp, Nannochloropsis gaditana
  misc_feature: TCTP promoter
cgtgcaggtgtacagattgaaggaaacaatggagatatctttggcagttgaaaaccgtgttcgaatcatgcttttctactctccaactgagacgaaatttatagcgccatgtcgcttctgactaccaggcttaggaaggcctcatcacaagctggatcggttcgaattaagcaggcactgaagccaagcttgcaagacagccaccttttaattccctcaaaacactttctcaattcagcccggtaaatatgccgattcacagcggccaagatagaggggaggttagcaagaatgttgcgatccctccccagtcgttgcctcgcacacaacctaggccttcacctttccatggaaaattgagaagtgaatattggttttcttacggcatatcagatgaaatcatgacccctaaacatgaagagctgcaggcaaaacacctgctctggacgagcacgatgaaatctcgagaacccgccgtacttcagttgatcccgcatgatgacggccgccattgaaataagccacctcactttattctagcaccgatttccaccgttgtgagggccgaacgaggacaatttcgtgcgaaacaagcacgaacacgcacacgattagtagtacagacgagcagatcgatggcatgcggcacggtctcgcgttctcggcgaccaggacaacggagcagagggaggcctgccgagttccgaggggcattttagtccaaaattgtgttgacacgtgaacaagtggcttgaaaagaggaaggaaatgcctgggtttcccttcgagagcgggaactcgcttgtgcgtcatcctagctacccatggtccctttgtgggggaggctgtttcgtcctaccgaatgtgtggcgctccatgcatcttctgcctcccaaaccaccaacatgagcacgcgaaggaaggagaaaaaagtggccgcaacgttctcttctcatatttattgtctcatcacaaacataggtacataatacaacaatc

SEQ ID NO: 40 - DNA, 317 bp, Nannochloropsis gaditana; identical to SEQ ID NO: 37
  misc_feature: EIF3 terminator

SEQ ID NO: 41 - DNA, 702 bp, Artificial Sequence
  Unknown
  misc_feature: TurboGFP gene codon optimized for N. gaditana
atgttggagagcgacgagagcggcctgcccgccatggagatcgagtgccgcatcaccggcaccctgaacggcgtggagttcgagctggtgggcggcggagagggcacccccgagcagggccgcatgaccaacaagatgaagagcaccaaaggcgccctgaccttcagcccctacctgctgagccacgtgatgggctacggcttctaccacttcggcacctaccccagcggctacgagaaccccttcctgcacgccatcaacaacggcggctacaccaacacccgcatcgagaagtacgaggacggcggcgtgctgcacgtgagcttcagctaccgctacgaggccggccgcgtgatcggcgacttcaaggtgatgggcaccggcttccccgaggacagcgtgatcttcaccgacaagatcatccgcagcaacgccaccgtggagcacctgcaccccatgggcgataacgatctggatggcagcttcacccgcaccttcagcctgcgcgacggcggctactacagctccgtggtggacagccacatgcacttcaagagcgccatccaccccagcatcctgcagaacgggggccccatgttcgccttccgccgcgtggaggaggatcacagcaacaccgagctgggcatcgtggagtaccagcacgccttcaagaccccggatgcagatgccggtgaagaataa

SEQ ID NO: 42 - DNA, 822 bp, Nannochloropsis gaditana
  misc_feature: 4AIII promoter
ggcataaaggacggcaaggaaagaaaagaaagaaagaaaaggacacttatagcatagtttgaagttataagtagtcgcaatctgtgtgcagccgacagatgctttttttttccgtttggcaggaggtgtagggatgtcgaagaccagtccagctagtatctatcctacaagtcaatcatgctgcgacaaaaatttctcgcacgaggcctctcgataaacaaaactttaaaagcacacttcattgtcatgcagagtaataactcttccgcgtcgatcaatttatcaatctctatcatttccgcccctttccttgcatagagcaagaaaagcgacccggatgaggataacatgtcctgcgccagtagtgtggcattgcctgtctctcatttacacgtactgaaagcataatgcacgcgcataccaatatttttcgtgtacggagatgaagagacgcgacacgtaagatcacgagaaggcgagcacggttgccaatggcagacgcgctagtctccattatcgcgttgttcggtagcttgctgcatgtcttcagtggcactatatccactctgcctcgtcttctacacgagggccacatcggtgcaagttcgaaaaatcatatctcaatcttcagatcctttccagaaacggtgctcaggcgggaaagtgaaggttttctactctagtggctaccccaattctctccgactgtcgcagacggtccttcgttgcgcacgcaccgcgcactacctctgaaattcgacaaccgaagttcaattttacatctaacttctttcccattctctcaccaaaagcctagcttac

SEQ ID NO: 43 - DNA, 200 bp, Nannochloropsis gaditana
  misc_feature: Bidirectional terminator 5
gggtgggaaggagtcggggagggtcctggcagagcggcgtcctcatgatgtgttggagacctggagagtcgagagcttcctcgtcacctgattgtcatgtgtgtataggttaagggggcccactcaaagccataaagacgaacacaaacactaatctcaacaaagtctactagcatgccgtctgtccatctttatttcct

SEQ ID NO: 44 - DNA, 20 bp, Nannochloropsis gaditana
  misc_feature: Target sequence for cpSRP54 gene
ggccacgcccttgctccgtc

SEQ ID NO: 45 - DNA, 2400 bp, Artificial Sequence
  Unknown
  misc_feature: HygR cassette
tccacagcccgaacccatgagagagaatcataatcaaagatgagccagccacgaagctaccggagaattctgtaagaaaaatgtttaaagttgaaaatgctaacagtgaagtgatatccttttttaatggagtgttgaggtgaagtctagcatcgtaggggaaaacaggattctgtgtcttccattctactccttgataaagcgaagaaatccgacaaaaccaaagagattgttcaagtttaagatttgtaagcgtacaactatgaacttcttctctttgtaggcctgagtggtcgtatgcatacgattcatgaagtgaatcagtatcgctggattttgcttaggagtaaagcacaactaagaaaatatgctgcctggcaggcatcctgagacatgaggcaagcgacgtagcaattgaatcctaatttaagccagggcatctgtatgactctgttagttaattgatgaaccaatgagctttaaaaaaaaatcgttgcgcgtaatgtagttttaattctccgccttgaggtgcggggccatttcggacaaggttctttggacggagatggcagcatgtgtcccttctccaaattggtccgtgtggtagttgagatgctgccttaaaattctgctcggtcatcctgccttcgcattcactcctttcgagctgtcgggttcctcacgaggcctccgggagcggattgcgcagaaaggcgacccggagacacagagaccatacaccgactaaattgcactggacgatacggcatggcgacgacgatggccaagcattgctacgtgattattcgccttgtcattcagggagaaatgatgacatgtgtgggacggtctttacatgggaagagggcatgaaaataacatggcctggcgggatggagcgtcacacctgtgtatgcgttcgatccacaagcaactcaccatttgcgtcggggcctgtctccaatctgctttaggctacttttctctaatttagcctattctatacagacagagacacacagggatcatggggaagaaaccggaactgaccgctacgtccgtggagaaattccttattgagaagttcgactctgtctccgacttgatgcaactgagcgagggagaggagagtagggcgttctcgtttgacgtagggggtcggggatacgtgttgagggttaatagttgtgcggacgggttctacaaggatcggtatgtctaccgtcatttcgcctccgccgctctccccataccagaggtactggacattggggagtttagcgaatctctcacgtactgcatctcgcgccgagcccagggagtgacgttgcaagatctgcccgaaactgaattgcctgccgttttgcaacccgtggccgaggccatggacgcgatcgctgccgcagatctgtctcagacgtccggctttggaccttttgggccccagggcatcgggcagtacacgacctggcgagacttcatctgcgccattgccgatcctcacgtctatcattggcagacagtcatggatgacaccgtgtctgcatccgtggcccaagcactggacgaactcatgttgtgggccgaggattgccctgaggtcaggcacctggtgcacgcggatttcggcagcaataacgtacttacagacaatggtcggattactgctgtcatcgactggtccgaagcgatgtttggtgatagccaatacgaagtggcgaacatattcttctggcgtccctggttggcgtgcatggagcagcagacacgctactttgaacggaggcacccggagctggccggctccccacgactccgcgcctatatgttgcgtatcggactcgatcagctttaccagtctctcgtcgacggcaacttcgacgacgccgcgtgggcgcagggccgctgcgacgcgatagtccgcagcggggctgggacggtgggtcggacccaaatcgcacgccggtcggctgcggtgtggacagacggctgtgttgaggtgcttgcggactcgggcaaccgtaggccgagcacccgaccgcgtgcaaaggagtgattgaatcattgaatgaaccattgtgtgcagaatcgatttcgggagtgttgccaacacaagaaatatgcccagggttgtgtagaagtttgcgtgaatgtgatgaagggaagccatacgctgaattatcgtgacgtgtgtgagacgaagtgtcacatcatacacccaatttgagaagctgtacctattagaagaatttgtgagatacattaaaccccttttggtacgtggtataattgttatttgggaagctgtaaacacgcagatcgttcctgagattgtcaattacttttgtggtgtttcctaaaggccgcatcactgcccgaatcgagttgatggcccgcaaa

SEQ ID NO: 46 - DNA, 1029 bp, Artificial Sequence
  Unknown
  misc_feature: Hygromycin resistance gene, codon optimized for Nannochloropsis
atggggaagaaaccggaactgaccgctacgtccgtggagaaattccttattgagaagttcgactctgtctccgacttgatgcaactgagcgagggagaggagagtagggcgttctcgtttgacgtagggggtcggggatacgtgttgagggttaatagttgtgcggacgggttctacaaggatcggtatgtctaccgtcatttcgcctccgccgctctccccataccagaggtactggacattggggagtttagcgaatctctcacgtactgcatctcgcgccgagcccagggagtgacgttgcaagatctgcccgaaactgaattgcctgccgttttgcaacccgtggccgaggccatggacgcgatcgctgccgcagatctgtctcagacgtccggctttggaccttttgggccccagggcatcgggcagtacacgacctggcgagacttcatctgcgccattgccgatcctcacgtctatcattggcagacagtcatggatgacaccgtgtctgcatccgtggcccaagcactggacgaactcatgttgtgggccgaggattgccctgaggtcaggcacctggtgcacgcggatttcggcagcaataacgtacttacagacaatggtcggattactgctgtcatcgactggtccgaagcgatgtttggtgatagccaatacgaagtggcgaacatattcttctggcgtccctggttggcgtgcatggagcagcagacacgctactttgaacggaggcacccggagctggccggctccccacgactccgcgcctatatgttgcgtatcggactcgatcagctttaccagtctctcgtcgacggcaacttcgacgacgccgcgtgggcgcagggccgctgcgacgcgatagtccgcagcggggctgggacggtgggtcggacccaaatcgcacgccggtcggctgcggtgtggacagacggctgtgttgaggtgcttgcggactcgggcaaccgtaggccgagcacccgaccgcgtgcaaaggagtga

SEQ ID NO: 47 - DNA, 1000 bp, Nannochloropsis gaditana
  misc_feature: EIF3 promoter
tcataatcaaagatgagccagccacgaagctaccggagaattctgtaagaaaaatgtttaaagttgaaaatgctaacagtgaagtgatatccttttttaatggagtgttgaggtgaagtctagcatcgtaggggaaaacaggattctgtgtcttccattctactccttgataaagcgaagaaatccgacaaaaccaaagagattgttcaagtttaagatttgtaagcgtacaactatgaacttcttctctttgtaggcctgagtggtcgtatgcatacgattcatgaagtgaatcagtatcgctggattttgcttaggagtaaagcacaactaagaaaatatgctgcctggcaggcatcctgagacatgaggcaagcgacgtagcaattgaatcctaatttaagccagggcatctgtatgactctgttagttaattgatgaaccaatgagctttaaaaaaaaatcgttgcgcgtaatgtagttttaattctccgccttgaggtgcggggccatttcggacaaggttctttggacggagatggcagcatgtgtcccttctccaaattggtccgtgtggtagttgagatgctgccttaaaattctgctcggtcatcctgccttcgcattcactcctttcgagctgtcgggttcctcacgaggcctccgggagcggattgcgcagaaaggcgacccggagacacagagaccatacaccgactaaattgcactggacgatacggcatggcgacgacgatggccaagcattgctacgtgattattcgccttgtcattcagggagaaatgatgacatgtgtgggacggtctttacatgggaagagggcatgaaaataacatggcctggcgggatggagcgtcacacctgtgtatgcgttcgatccacaagcaactcaccatttgcgtcggggcctgtctccaatctgctttaggctacttttctctaatttagcctattctatacagacagagacacacagggatc

SEQ ID NO: 48 - DNA, 27 bp, Artificial Sequence
  Unknown
  misc_feature: Synthetic
  misc_feature: 5'ID sequence
tccacagcccgaacccatgagagagaa

SEQ ID NO: 49 - DNA, 27 bp, Artificial Sequence
  Unknown
  misc_feature: Synthetic
  misc_feature: 3'ID sequence
gcccgaatcgagttgatggcccgcaaa

SEQ ID NO: 50 - DNA, 20 bp, Nannochloropsis gaditana
  misc_feature: 5' Primer, cpSRP54 locus
gcaggacaatgaaattgacg

SEQ ID NO: 51 - DNA, 20 bp, Nannochloropsis gaditana
  misc_feature: 3' Primer, cpSRP54 locus
gtggaggaacgtcagaggac

SEQ ID NO: 52 - protein, 516 aa, Nannochloropsis gaditana
  misc_feature: Ftsy polypeptide
MLQYHLLLLPLLMLPWAGWTQAAFVTPRVGGPRSYGDGRKYRVGVPFYSSIDEVDSPIYTTASRSRRQGESHMMVFDFIRKRAEEGIQQVQNIATKTAEGKFVEALGDTASYVKKRQEIDAENLAKLQEGLAKSRQRLMGDLDVIFGVSEDVGLTKTLDKLEEVLMMSDIGAATTGEIIDDLRMVAKAEKLEPDDVKSVLRLRLIEALTAKDRSMQLKKEASAGNGKSYPRVLFVIGANGMGKTTTIGKIASRLKNEANQSVLVAACDTFRAAAVDQLEEWTVRAGVDIHRPGEGQTKPAPVLEEAISKAIEGDYDVLIVDTSGRLSNNVALNEELKKLKRTIADGIPGGPHETLLVLDGAVGRNGVDQAKVWNREVGITGLVITKLDGTARGGVVVSIVRDVGVPVKLIGVGEGIDDLRDFNPEDFVDALLGYEPEQVLALEARLQDMVQGKLIKPKRGVIVRSEGGGRDKNMDADDISDRMRRKVQGRGGQGGSSSQRGGGKGGKSGGGKKKRR

SEQ ID NO: 53 - DNA, 1551 bp, Nannochloropsis gaditana
  misc_feature: Encodes Ftsy polypeptide
atgttgcagtatcacctcctcctcctacctctcctgatgctgccttgggcaggatggactcaagctgcattcgttactccaagagttggaggcccaagatcttatggtgatggaagaaaatacagagtcggtgtgccattctactcgtcaatcgacgaggtagacagtcctatctacaccacggcatcacgatccagaaggcaaggtgaaagccacatgatggtattcgattttattcgaaagcgggcagaagagggaatacaacaagtacaaaacatcgctactaaaactgcggaggggaagtttgtggaagctctaggcgacacagcctcctacgtcaaaaagcgacaggaaatcgacgctgagaaccttgcgaagcttcaagaaggcttagcaaagagcaggcagcgtctgatgggggacttggatgtgatttttggtgtgagcgaggatgtgggcctcacgaagactttggataagctggaggaagtgctgatgatgtcggacataggggcggccacgacgggtgaaatcatcgacgacctccgcatggtcgccaaggccgagaaactcgagcctgacgacgtcaagtctgtcctccgtttgcgtttgatcgaggcgttgacggccaaggataggagtatgcagttgaaaaaggaagcgtccgcggggaatggaaagagctaccctcgtgtcctcttcgtcatcggtgcgaacgggatgggcaagacgacgacgatcgggaagatcgcctcccgcctcaaaaatgaagcgaatcagagtgtgctggttgccgcctgtgacacttttcgcgccgccgctgtcgaccagctggaggagtggacggtgcgagccggcgtggacatccaccggccaggggaagggcagacgaaacccgcgcccgtgctggaagaggctatcagtaaggcgatcgaaggagactacgacgtgctgattgtggacacatctgggcggctttcaaataacgtggccttgaacgaggagctcaagaagttgaaaaggaccatcgcggacggcatccctggtggcccgcatgagaccctactcgtcttagacggcgccgtgggcaggaatggggtagatcaggcaaaggtctggaatcgagaggttggaatcacggggttggtcatcacgaaacttgacggcacggccaggggaggtgtggtggttagcatcgtgagggacgtgggcgtccctgtgaagctcattggagtgggcgaggggattgatgacttgcgggatttcaatccagaggattttgtggatgctttgttgggatatgagcctgaacaggtgctggccttggaggcccggcttcaagacatggttcaaggcaaacttatcaagccgaagagaggggtaattgtacgctctgaaggtggtggacgcgataagaatatggatgcagacgatatcagcgacaggatgagacggaaagtccaaggacgggggggccagggcggttcctcctcgcagcgtggagggggaaaaggaggaaaaagcggtggtggcaagaaaaagaggcggtaa

SEQ ID NO: 54 - DNA, 19 bp, Nannochloropsis gaditana
  misc_feature: Ftsy gene target sequence
ggcaggggaaagattaatg

SEQ ID NO: 55 - protein, 489 aa, Nannochloropsis gaditana
  misc_feature: ALB3 polypeptide
MPQPFFWSCREQCCDPCLQHSHRSELSYLFDFFHSNRMVMRTHQREMWRQQQCLGRRLGSCIFCLLMASLLFTSEVVTAFVPVATRRPDLLHVSRPPFPSRATPGTRALRMVLQPHDVVTHLDPAWLSHVFQGVADAAVTSLDATNAAVDATTDAAAKEPGFFDKFVNTVMGAIEGVHSELVSLGVPGAYGLAIILFTAGVKLALLPVTYKQMESAQRMQALAPKAKELKDKYGKNKALLNQLTAKLYEDAEVNPLAGCLPALAQIPIFIALYRSLINLAGNSDFNEPFLWLPSLAGPLYGQARGTDWLFKNWVDGVPALGWHDTIAFLTIPVILILTQSISQRLLTPPSDDPKTAQTQRVLKYLPIMVGYFSLSVPSGLGVYWITNNLISTAISISIKEKFAKQPIVIDVDVDPEDLGYDPSTVAMGFEEMMAEATRNALPSEQPKRDRPTPSSLLKASESVVAEEGGKRDEEAGRVGEEREKAGVEA

SEQ ID NO: 56 - DNA, 1470 bp, Nannochloropsis gaditana
  misc_feature: Encodes ALB3 polypeptide
atgccccaaccctttttttggtcttgccgcgagcagtgctgtgatccgtgcctgcaacattcacatcggagcgaactctcatatttgttcgattttttccattcaaacaggatggtcatgcggacgcatcagcgtgagatgtggcgtcagcagcaatgtctgggtagaagactagggtcatgtatattctgtctcctgatggcatcccttttgtttacttccgaggtggtcacagcatttgtgcccgtcgccacgcgtcggcccgacctcctccacgtctctcgccccccatttccttcgagagccacgccaggtaccagagctttgcgcatggttttacagccgcacgatgtggtgacgcacctggacccagcgtggctttcccacgtctttcagggcgtggcagatgcggccgtgacttctttggatgcgacaaatgccgcggtggacgccaccaccgatgccgccgcgaaggagccgggcttcttcgataaattcgtgaacacggtcatgggcgcgatcgagggtgtgcacagtgaactggtgtcgctcggcgtccctggcgcctacggcttggccatcatattgttcaccgcgggcgtcaaactggccctgcttcccgtcacctacaagcagatggagtcagctcagcgtatgcaggccctagcgcccaaggcgaaggagctcaaggacaagtacgggaagaacaaggcgctcctgaaccagctgaccgccaagctctacgaggacgcggaggtgaaccctctcgccggctgccttcccgccctcgcccaaattcccattttcattgccctctaccgctccctgatcaaccttgcggggaacagcgacttcaacgagccctttctctggctgccgagtctggccgggcctctctacggccaagcccgaggcacggactggctcttcaaaaactgggtggacggcgtcccggccctgggctggcacgacacaatcgccttcctcaccatccccgtcatactgatcctcacgcagtctatctcccaacgactgctcaccccgcccagcgacgaccccaagaccgcgcagacccagcgcgtcctcaaatatctgcccatcatggtcgggtacttctctctgagcgtgccctccggcctgggtgtctactggatcaccaacaatttgatctccacggccatctcgatcagcatcaaggagaagttcgccaagcagccgatcgtgatcgacgtggatgtggacccggaggacttgggctacgacccctccacggtggccatgggcttcgaagagatgatggcggaggcgacgcgcaacgcgcttccaagcgagcagcccaagcgggatcgaccgacgccatcctcccttttgaaagcgtcagagagtgtcgtggctgaggagggggggaagagggacgaggaggccggccgcgtgggggaggagagagaaaaagcgggcgtggaggcctga

SEQ ID NO: 57 - DNA, 20 bp, Nannochloropsis gaditana
  misc_feature: ALB3 gene target sequence
gggaaagccacgctgggtcc

SEQ ID NO: 58 - protein, 562 aa, Nannochloropsis gaditana; identical to SEQ ID NO: 30
  misc_feature: Cytosolic SRP54 polypeptide

SEQ ID NO: 59 - DNA, 1689 bp, Nannochloropsis gaditana; identical to SEQ ID NO: 29
  misc_feature: Encodes Cytosolic SRP54 polypeptide

SEQ ID NO: 60 - DNA, 20 bp, Nannochloropsis gaditana
  misc_feature: Cytosolic SRP54 gene target sequence
ggccagcgggggcatctgca

SEQ ID NO: 61 - DNA, 5607 bp, Artificial Sequence
  Unknown
  misc_feature: Cas9 gene codon optimized for Parachlorella and including Parachlorella introns, FLAG tag NLS, peptide linker
atgcccaagaagaagcggaaagtcggggactacaaggacgacgatgacaaactggagcctggggagaagccctataagtgtcctgagtgcgggaagagcttcagccaatctggagcactgacaaggcaccagaggacacatacacgcgacaagaagtacagcatcgggctggatatcgggaccaattctgtgggatgggccgtgattaccgacgagtataaggtgcccagcaagaagttcaaggtgctggggaacacagaccgccacagcattaagaagaacctgatcggggcgctgctgtttgattctggagagacagcagaggcaaccgtgagtgagaacagttttcagatcgaatagcacccccccgcctctgcagcagtcgcataccggctgcagtaatagcttggttcaacggcgacctgaacaagtactgtagtttctatgcatacgaactttatcgaatagaatcacgcttgggtatcgatcataccttagcgctcaatttcattggctgctacagaccatattttcctcttcacttgttgcagcgcctgaaaagaacagcaagaaggcgctacacccgccgcaagaataggatttgctacctgcaagagatcttcagcaacgagatggccaaggtggacgacagcttcttccatagactggaggagtcgttcctggtggaggaggataagaagcacgagaggcaccccatcttcggtgagaagagtttggctaccaaatctatcttttcatatcacatataccgcctgatattctgaggtggtggcttttgtctttttctttcagtatttttcttcgttgggaacctaccgcgagggcattcattgtggcggatctgtaagtgcgaccaggctgtatccaatattttttcctatcgcagggaacattgtggatgaggtggcctaccacgagaagtaccccacaatctaccacctgcgcaagaagctggtgagaatctctgcttgtcgaatgtgtccagttgtgtcttgaatcctggcaagatgttcttttcaccatccgtcctgcaaaagtgtcagaagtagcatctctcgatcgcgttgtcacttcaacgcctccgcaactccccccgttgtgaatcctgtggtcatggctcagcttttcagatctctacctgcatgttgtttgcctgtctcagtcctgcctgcacaaatcatcgcccttgtttactccttgcaatcacggattgtgtgcaggtggacagcacagataaggccgatctgaggctgatctacctggcattggcccacatgatcaagtttagggggcacttcctcatcgagggggatttgaaccccgacaacagcgatgtggacaagctgttcatccagctggtgagtggagggctggggtttgggggtggggggtggggagggaggcacggatggtgttttctcatgtccaaccgtggttcatgcaaccgaacagcagtttcacaagatggttccaacagggtgctccatttctccctgacaaaacctcgtgcggtccatctggtatagctgggttagtagggggttgtgggctgtccacagtcagtgcgaagcaggctctattgagcgtgtgctagtgtgtgctgtgctgattggcattttgttgggccgagtgttaggattagggtaaatcaccctaattaaccttacataataggactgtatgcaaatttgttttccaaaaactctacccagcgtggtcagactgcatgcactgtggagcatgcatggggctgaccctgttgatcctgctcattctgcttcctccaggtgcagacctacaaccagctgtttgaggagaaccccatcaacgcatctggggttgacgcaaaggccattctgtctgcaaggtaggtgcaggaagaagtgaatgatgcacacatggtggaatcgtgatacaagcagcagcaagtgttggaccaagacatgtgcgtgctttgctgctgccaagctggcactgcaccaggtcgtgcattgatctgcacatttgatatactgtgagagtcagacgacgtcctttcagagcctgtgtgtgattctccaggggttaacacgagtttcctttctgccagtgagtcaccctctcgctgctcgctcctggtgcaggctgagcaagtcaaggagactggagaacctgatcgcccaattgcctggagagaagaagaacgggctgttcgggaacctgatcgcattgtctctggggttgacccccaacttcaagagcaacttcgacctggcagaggacgcaaaactgcagctgagcaaggacacctacgacgatgatctggacaacctgctggcccagattggagatcagtacgcagacctgttcctggcagccaagaatctgagcgacgcaattctgctgagcgacattctgcgcgtgaacaccgagatcaccaaggcacctctgagcgcaagcatgatcaagaggtacgacgagcaccaccaagacctgacactgctgaaagcactggtgagacagcagctgcctgagaagtacaaggagatcttcttcgaccagagcaagaacgggtacgctgggtacattgatggaggagcaagccaagaggagttctacaagttcatcaagcccatcctggagaagatggacgggacagaagagttgctggtgaagctgaatcgcgaggatctgctgaggaagcagaggacattcgacaatgggagcatcccacaccagatccatctgggagagctgcacgcaattctgaggagacaagaggacttctacccgttcctgaaggacaatcgcgagaagatcgagaagatcctcacgttccgcatcccgtactatgtgggacctctggcaagggggaactctagatttgcctggatgacccgcaagagcgaggagacaattacaccctggaacttcgaggaggtggtggataaaggggcatctgcacagagcttcatcgagaggatgaccaacttcgacaagaacctgcccaacgagaaggtactgcctaagcattcactgctgtacgagtacttcaccgtgtacaacgagctgaccaaggtgaagtacgtgacagaggggatgaggaagccagcatttctgagcggagagcaaaagaaggccatcgtggatctgctgttcaagaccaaccgcaaggtgaccgtgaagcagctgaaggaggactacttcaagaagatcgagtgcttcgacagcgtggagatttctggagtggaggaccgcttcaacgcatctttggggacataccacgacctgctgaagatcatcaaggacaaggacttcctggacaacgaggagaacgaggacatcctggaggacattgtgctgacactgaccctgttcgaggatagggagatgatcgaggagcgcctgaagacatacgcacacctgtttgacgacaaggtgatgaagcagctgaagaggaggcgctatactggatggggaaggctgtcaaggaagctgattaacgggatccgcgacaagcagagcgggaagacaattctggacttcctgaagagcgacgggttcgcaaaccgcaacttcatgcagctgatccacgacgatagcctgaccttcaaggaggacatccagaaggcccaagtgtctggacaaggggatagcctgcatgagcacatcgcaaatctggctgggtcacccgcaatcaagaagggaattctgcagaccgtgaaggtggtggatgagctggtgaaggtgatgggaaggcacaaacccgagaacatcgtgatcgagatggcaagggagaaccagacaacccagaagggacagaagaactctagggagcgcatgaagcgcatcgaggagggaattaaggagctgggaagccagatcctgaaggagcatcctgtggagaacacccaactgcagaacgagaagctgtacctgtactacctgcagaacgggagggacatgtacgtggatcaagagctggacatcaaccgcctgagcgactatgacgtggaccacattgtgcctcagtcgttcctgaaggacgacagcatcgacaacaaggtgctgacaaggagcgacaagaatcgcggaaagagcgacaacgtgccttcagaagaggtggtgaagaagatgaagaactactggcgccagctgctgaacgcaaagctgattacacagcgcaagttcgacaacctgaccaaggcagagaggggaggactgtcagaactggataaggccgggttcatcaagaggcaactggtggagacacgccagatcacaaagcatgtggcccagattctggacagccgcatgaacaccaagtacgacgagaacgacaagctgatccgcgaggtgaaggtgattaccctgaagagcaagctggtgagcgactttcgcaaggacttccagttctacaaggtgcgcgagatcaacaactaccaccacgcacacgacgcctacctgaatgcagttgtgggaacagccctgatcaagaagtaccccaagctggagagcgagttcgtgtatggggactacaaggtgtacgacgtgcgcaagatgatcgccaagtctgagcaagagatcgggaaggcaaccgccaagtacttcttctacagcaacatcatgaacttcttcaagaccgagatcaccctggccaatggggagattaggaagagacccctgatcgagaccaacggagagactggagagatcgtgtgggataaggggagggactttgcaacagtgcgcaaagtgctgagcatgcctcaagtgaacatcgtgaagaagaccgaggtgcagactgggggattctcaaaggagagcattctgcccaagcgcaacagcgataagctgattgcacgcaagaaggactgggaccccaagaagtatggggggtttgatagccccaccgtggcatattctgtgttggttgtggccaaggtggagaaggggaagagcaagaagctgaagagcgtgaaggagctgctggggatcaccattatggagaggagcagcttcgagaagaaccccatcgacttcctggaggcaaaggggtataaggaggtgaagaaggacctgatcatcaagctgcccaagtacagcctgttcgagctggagaatgggaggaagaggatgctggcatctgctggagaactgcagaaggggaatgagttggcactgcctagcaagtacgtgaacttcctgtacctggccagccactacgagaagctgaagggatcacccgaggacaatgagcagaagcagctgtttgtggagcagcacaagcactacctggacgagatcatcgagcagatcagcgagttcagcaagcgcgtgattctggcagacgcaaacctggataaggtgctgagcgcctacaacaagcaccgcgataagcccattcgcgagcaagcagagaacatcatccacctgttcaccctgaccaacctgggagcacctgcagcattcaagtacttcgacaccaccatcgaccgcaagaggtacacaagcaccaaggaagtgctggacgcaaccctgattcaccagagcattactgggctgtacgagacacgcatcgacctgtcacaactgggaggggactga

SEQ ID NO: 62 - DNA, 588 bp, Parachlorella sp.
  misc_feature: RPS17 promoter
caacacctagttggtaaataccgttgctgatattgctctgtaccagtaaaagagggctgcgatgagcgtttttagtgcacttcttcaacacggaatatttttcacaaattggtatgagaaccaattttgcaaaatgttcgccctgtaaagtatcgctctgggacgatcagcttgacgtaattgtaggcgaaaagggcgttcaaagtgcagctttatgtatgaacgtcataaaatataaagcatagcacaatcactgatagaaaatatttgtgcgcattaaaactctcacttctgttgcggatacaacgacggaaatgagaagcttgtgtaagaagcaattcaagttttcattttgtcatctaaggtgtgatcctccgatattcattaccgaatgctgatctgagttggaaagatggcaatatttagctgtgcacactttgacctccaggccttggcgggaatttagtattctagctttcctattggaacgataggccagccaagtctccagcttgtatacgctacaccagcagacatgctctcaatttagctgacagtgtcttcatatttgtattatctgttgtgtct

SEQ ID NO: 63 - DNA, 455 bp, Parachlorella sp.
  misc_feature: RPS17 terminator
ggtgcgaatagtgcttcagtaaaaaagtagcaacttggtgcaatatcgtcagggtcgtgtggtctgctcgccagcaagttttttggcacaggagagcgctttttccgagtaccgccaaagttcaagcatgtgctgtgattcgctgttgcctcttatgataattgctcaaagtttccaagcattctatgtccaccctgcaccactaagttgtatggtgcttattctgcaggggatgattcatggtgcctaaaaattttgtgctgctgtcgcgtctgttttctgtcgcagtttagtgaatgtaactccaaataccaaacttttcatcacaatcatattgatgcctttgtaagtgaattacagcgttttttgccataaaaagaagtaccgtgacattggggtcgtcataacaagaagctttatgaacaagcagcttgatctacgagacttatacataa

SEQ ID NO: 64 - DNA, 2691 bp, Artificial Sequence
  Unknown
  misc_feature: Blasticidin resistance gene from Aspergillus terreus codon optimized for Parachlorella and containing Parachlorella introns
atggcaaaacctctctcccaggaagagtctaccctgattgaaagggcaacagcaaccatcaacagcattcccattagcgaggactactctgttgtgagttctgagaagctgattgttgtttaacttctttgaaagctttatcgaagattctgcaagcgatgaacattgcttgtcaagaccgagagctgcatgcccacttgacatccagctttgaacggctcttcatgtttgatttgtttctgattgtaggcatctgcagcattgagctctgatggaaggatctttacaggagtgagtgcagcgtcagctgtggcagttgttggctttcgtctcagtcagtagtttgctgggattgattatggagggcacagttgcaattttgagttgcacgttgcgacaagcgtgttgacaaagcgtggtcaagccggccagtcttgccggtggcgggtggcttggtctaacttccgctctacggcaatcgttttgttcatggttacggggctggcgtgccagaaagtcctggtcagccaccctcgcttcaaagccgtagcccaacaactttgcgaatatgttcgatttgcaggtgaacgtgtaccactttacaggaggaccttgtgcagaattggtggtgttaggtacagctctgcgtgcaacaggttgcaagatgcagcgcaggtcttccctggtcaaacgatgtatgcagagttgagaggcacttgagctgggtgaatggcgtgggctcgtaggtagtgtgcagggcaggaagggcagccaattttggagttgtggtccggtgtcgttgcttcgagccttattaggactcttgctcatcaaagcgttagttgtgaataagttgatctgaaaggatgttatgtacagcaagcagcagcagttaagagtctggggagtagctgcacagggcgaggtgtcaagatgggaagggtcctgcctccttatgtgtttttccctgtaggggaggaagcctcttatgggcaatggttgggcatattttccagccagcccttctttctataggggccagggtgggcccagctcgtcttggcttccaccaccaggagagtgagggcattgaagggccataaatagtcctcccatctacgtgcaccagagggtgtcgtctaggctgtgcatgccacgaggggaaggagccaagaatgagtgtatgggttgttttcatgtttaggctgggataaaactgttttcaattgcgcctgccgggtgaaaaccacagcagcatcagcaagcttggagaaggccagcccgcccagcacaggctcacgttcccactcaggcggtcagtcgggcgggggtgtgagtcaggcaggcgagggtgtctgtgcctgacatcagcacctctgcttagccactgcagcccctggagcagggtagggcgtcatttgcagcaatcacctgctgcctcacacgtcgcagcttggaatttcaacgaccatcagcgctggggttgttgagggatcatagcagattttggtgcagcctggttgtcatgctctttgtggaatggcctctatgttcgagcaattcgttggatgttgaggtgcttggggacagagagtcgaatgatgggccagggtcaaacatgcgagcgtttggctgagtcagcggtttttgctggtcactttttcttttgtttcttatttaggtttgatggatgtgttttgtgctgctgccctgaagctgcagcagcgtgtctgccctgcgctactgcgggcaccaaggctatgtgctggtgcactcggctgcgctgcacctgtgcacctcgcactccgtccagcctccatgcagcacacgtactcacggtgtcctcctgacctgtcgtacgctattccaaacttgctcttttgctgccgctgctctcgtacacaattgctgttgattatcgatatctaatcgagcgcctgctgactgaactccgcaggtacagcagctgcagcagcagcaggaaatttgacatgcattgtggcaataggtgggtgggctctgaaggaggaggagggagcgggtgattaaacagggcctgcatgaagaggagcaggggctgcgtggacagcagggggaaggtgcagaagggagggtcaagcggggttcaggtggctgtgggtttctgcacgagcagtgaaagaagctgtatccttccacctgcttccactggcgaaaggttgaaaacaggatgtcgcagctggaaagatgttgcgctgtcaagtgcaagccatggttgagggtatgcctgtgtgcatgtgcttcttaaagttactcctgttctatggttctgggtgcttgttgtttgtggtgcagggaacgagaatagggggattttgtcaccttgcggaagatgtagacaggtgttgttggatctgcatcccgggattaaggtgagggggcatgtaagcaatggcaggcaattcaagaacgaatcattgctgcaaatgctgggatggtatgcagctgaggtatctattgccttgtattttgtctcgcattgcatcggtggtgcgttctgtggcctgaggcacagttcttgctgtttgataagggttcgactgagttgtcgtgtgtgctgtgctgcaggcaatcgtgaaggattcagatgggcagcctacagcagtgggaattagagaactgctgccttctgggtatgtgtgggaaggataa

SEQ ID NO: 65 - DNA, 530 bp, Parachlorella sp.
  misc_feature: RPS4 promoter
ccaccatgggggaggtttgaagtgtgcgcctgatataatcatacacctaaaagcaccacttgctgattgtgaagggactatgtcgtttatgacgggacgttacgctggccgatggtttgaatttggacgctgtggtagaatgttatatggacgtaaaggttggcatattgaaaatcgtcttcgcaggcaaacttctagacgtgtgacccaccggtaaaacgacaagcgtggcgcgtcgattgcgctttgaacgtcgtttgttggactccagatgaacctcaaaatcaaagcggtgattgacgaaaatcaaatgacagcccgcaaaatttcatcagccttcggatcggattctcagaatctgattgtccctgctggctacatttatgaaatttcgtacattttggcagaaatgtcccaataccatagcactgccgcctgagctcacccgagcaatgcatactgggtacctcgcccatctcgccctctttccaagcccagtgctgttgtaatagccaaagggctcagtaaca

SEQ ID NO: 66 - DNA, 546 bp, Parachlorella sp.
  misc_feature: RPS4 terminator
gcatagcatcagcctgtggcagggttgtggtagggctgagtggcagggttaaaggggttgcctaccccacccctactctcatgacaccagcaacagcagcagctcatgcagtactcaaatcactgatgtcaatggtgtgacacatttggttaaggctgctttttaaagtgctgctttgggggcagtgactgtgcagagcttggagcgtatccccatgtaatcagaaccgacgagagttcggggcaacctttcatcttcacattttttgtgatcagctacagagtctgaaatcaaatagaggctgccatctaaacgcaggagtcacaacgaaggcgaaaactccaattgctgtactcaatgcactaagtgattgttcaatggataaatacactatgctcaattcatgccagcagagctgctccttccagccagctacaatggctttttccacgccttttgaagtatgaatgttcagcttgctgtgcttgatgcatcaccataaacacaattctacaacatttcatgccaacaacagtacgggctttc

SEQ ID NO: 67 - DNA, 572 bp, Parachlorella sp.
  misc_feature: ACP1 promoter
agtttgcatagttaagtatgctggctattgcagtaccttatatgcaaacaagtgctcaatctgtttcatcattgtctgtgggcaaattgcctgccaatattctccagttattgcctgttgtttcaaatgattgaaattggaagttgtattgctctacatttttgacttgtgattttttcatttgttgatatctgacaactgtgaactgcactgaacttgctgtgcttataaatgcatttttttgttttgggccacgttgattccttgtgatactttcctgctatcaaaccaaaaatatactctcatgactgacgtgcaacaaatgcatggaagctttcaacgttacgacagctgcttgccccccatcagctattctacatgtgtaacctaccttgcatggccaccacaacgctactgcatgcaagatctggcgcaactggatgtcccaatagtagaagtatccggattatctccgagagttttacatatgtaatcgacgccatttctgtcatcaactataaatccattgctcctgcatttctggcactgacattctaccacaagcaatacca

SEQ ID NO: 68 - DNA, 869 bp, Parachlorella sp.
  misc_feature: ACP1 terminator
gcagcagcttgttatgccttccccatgggcatcagcatgctgcaagctgtctagatatccagctttcagtggaggttgagcgagggtcagcagcggttccctggcgatggcggtcagcttttctggaagccttcactaggactgcgcccagcgcatgtgacgccaatcgaacttgtgtgcaaggccaaattttgtgaccctgtgctgcacttcatgtattcaagaattgagaagaaatttcattgctgcccttctttcactttaatttccatccctggatccacctcccaccattgtggttgatgggtaggggttttgggtaggtgcagttcgttgtgcacgttgacatgtgtaacggtgagcaaaggaattgctgggcaagtagctattgcagcttaagggcatggtgaaacacttgtgctgtatttacagaggaagccagacaggtaaggagtgtgtggcagcttggaacaggagggctggtcgcaacaagtatgcatatcccatgattgttgacataagagcagcaggtgcatattgccagcctttgtgaaagtggattgaaaatcgattagttggtgtgatagctgaggctaggcactgccaacctgcagtgaaatgaggctccaagaccgggtaataatacaggcaatcgaatccagttgaaattacggcgattaaatccaagcgagcgttgtaagaacatctgcacctgtctgaagtagtgagcggataatgagcattgcttgccttctatcactatacctgacagttacgtgtcacacactctcaagcacaacacacagcggcaaagttacttgctaaacctcacagtcaagctgaaaataaaggctaaattacgtgagacc

SEQ ID NO: 69 - DNA, 1707 bp, Parachlorella sp.; identical to SEQ ID NO: 1
  misc_feature: Chloroplastic SRP54 coding sequence

SEQ ID NO: 70 - DNA, 2667 bp, Parachlorella sp.
  misc_feature: Bleomycin resistance gene codon optimized for Parachlorella and containing Parachlorella introns
atggccaaactgacatccgctgttcctgtgttgacagcaagagatgttgcaggtgcagtggagttttgtgagttctgagaagctgattgttgtttaacttctttgaaagctttatcgaagattctgcaagcgatgaacattgcttgtcaagaccgagagctgcatgcccacttgacatccagctttgaacggctcttcatgtttgatttgtttctgattgtagggacagatagactggggtttagcagggactttgtggaggacgattttgcaggagtggtgagggatgatgtgacactgtttatctcagcagtgcaggatcaagtgagtgcagcgtcagctgtggcagttgttggctttcgtctcagtcagtagtttgctgggattgattatggagggcacagttgcaattttgagttgcacgttgcgacaagcgtgttgacaaagcgtggtcaagccggccagtcttgccggtggcgggtggcttggtctaacttccgctctacagcaatcgttttgttcatggttacggggctggcgtgccagaaagtcctggtcagccaccctcgcttcaaagccgtagcccaacaactttgcgaatatgttcgatttgcaggtggtgcccgataatacactggcatgggtttgggtgagaggtacagctctgcgtgcaacaggttgcaagatgcagcgcaggtcttccctggtcaaacgatgtatgcagagttgagaggcacttgagctgggtgaatggcgtgggctcgtaggtagtgtgcagggcaggaagggcagccaattttggagttgtggtccggtgtcgttgcttcgagccttattaggactcttgctcatcaaagcgttagttgtgaataagttgatctgaaaggatgttatgtacagcaagcagcagcagttaagagtctggggagtagctgcacagggcgaggtgtcaagatgggaagggtcctgcctccttatgtgtttttccctgtaggggaggaagcctcttatgggcaatggttgggcatattttccagccagcccttctttctataggggccagggtgggcccagctcgtcttggcttccaccaccaggagagtgagggcattgaagggccataaatagtcctcccatctacgtgcaccagagggtgtcgtctaggctgtgcatgccacgaggggaaggagccaagaatgagtgtatgggttgttttcatgtttaggctgggataaaactgttttcaattgcgcctgccgggtgaaaaccacagcagcatcagcaagcttggagaaggccagcccgcccagcacaggctcacgttcccactcaggcggtcagtcgggcgggggtgtgagtcaggcaggcgagggtgtctgtgcctgacatcagcacctctgcttagccactgcagcccctggagcagggtagggcgtcatttgcagcaatcacctgctgcctcacacgtcgcagcttggaatttcaacgaccatcagcgctggggttgttgagggatcatagcagattttggtgcagcctggttgtcatgctctttgtggaatggcctctatgttcgagcaattcgttggatgttgaggtgcttggggacagagagtcgaatgatgggccagggtcaaacatgcgagcgtttggctgagtcagcggtttttgctggtcactttttcttttgtttcttatttaggtttgatggatgtgttttgtgctgctgccctgaagctgcagcagcgtgtctgccctgcgctactgcgggcaccaaggctatgtgctggtgcactcggctgcgctgcacctgtgcacctcgcactccgtccagcctccatgcagcacacgtactcacggtgtcctcctgacctgtcgtacgctattccaaacttgctcttttgctgccgctgctctcgtacacaattgctgttgattatcgatatctaatcgagcgcctgctgactgaactccgcaggtttggatgaactgtatgcagagtggtctgaagtggtgagcaccaactttaggtgggtgggctctgaaggaggaggagggagcgggtgattaaacagggcctgcatgaagaggagcaggggctgcatggacagcagggggaaggtgcagaagggagggtcaagcggggttcaggtggctgtgggtttctgcacgagcagtgaaagaagctgtatccttccacctgctttcactggcgaaaggttgaaaacaggatgtcgcagctggaaagatgttgcgctgtcaagtgcaagccatggttgagggtatgcctgtgtgcatgtgcttcttaaagttactcctgttctatggttctgggtgcttgttgtttgtggtgcagggatgcaagcggacctgcaatgacagagattggagaacaaccttggggaagggagtttgcattgagagatcctgcaggtgagggggcatgtaagcaatggcaggcaattcaagaacgaatcattgctgcaaatgctgggatggtatgcagctgaggtatctattgccttgtattttgtctcgcattgcatcggtggtgcgttctgtggcctgaggcacagttcttgctgtttgataagggttcgactgagttgtcgtgtgtgctgtgctgcaggcaattgcgtgcactttgttgcagaagaacaggactga

SEQ ID NO: 71 - DNA, 32 bp, Artificial Sequence
  Primer AE596
tgcgacatgcagcttactaacctgctcgacat

SEQ ID NO: 72 - DNA, 28 bp, Artificial Sequence
  Primer AE597
atgggctccttgatgttgtccgccgtta

SEQ ID NO: 73 - DNA, 21 bp, Artificial Sequence
  Primer AE405
acccaaacccatgccagtgta

SEQ ID NO: 74 - DNA, 25 bp, Artificial Sequence
  Primer AE406
actgtatgcagagtggtctgaagtg